European Patent Application EP 4 218 799 A1, published August 2, 2023. Title: RSV F PROTEIN COMPOSITIONS AND METHODS FOR MAKING SAME. Applicant: GlaxoSmithKline Biologicals SA. Application EP, filed July 15, 2010. The sequence listing filed with the application follows.

SEQUENCE LISTING (112 sequences)

SEQ ID NO: 1 - protein, 574 aa, Human respiratory syncytial virus
MELLILKANAITTILTAVTFCFASGQNITEEFYQSTCSAVSKGYLSALRTGWYTSVITIELSNIKENKCNGTDAKVKLIKQELDKYKNAVTELQLLMQSTPPTNNRARRELPRFMNYTLNNAKKTNVTLSKKRKRRFLGFLLGVGSAIASGVAVSKVLHLEGEVNKIKSALLSTNKAVVSLSNGVSVLTSKVLDLKNYIDKQLLPIVNKQSCSISNIETVIEFQQKNNRLLEITREFSVNAGVTTPVSTYMLTNSELLSLINDMPITNDQKKLMSNNVQIVRQQSYSIMSIIKEEVLAYVVQLPLYGVIDTPCWKLHTSPLCTTNTKEGSNICLTRTDRGWYCDNAGSVSFFPQAETCKVQSNRVFCDTMNSLTLPSEINLCNVDIFNPKYDCKIMTSKTDVSSSVITSLGAIVSCYGKTKCTASNKNRGIIKTFSNGCDYVSNKGMDTVSVGNTLYYVNKQEGKSLYVKGEPIINFYDPLVFPSDEFDASISQVNEKINQSLAFIRKSDELLHNVNAGKSTTNIMITTIIIVIIVILLSLIAVGLLLYCKARSTPVTLSKDQLSGINNIAFSN

SEQ ID NO: 2 - protein, 574 aa, Human respiratory syncytial virus
MELLIHRSSAIFLTLAVNALYLTSSQNITEEFYQSTCSAVSRGYFSALRTGWYTSVITIELSNIKETKCNGTDTKVKLIKQELDKYKNAVTELQLLMQNTPAANNRARREAPQYMNYTINTTKNLNVSISKKRKRRFLGFLLGVGSAIASGIAVSKVLHLEGEVNKIKNALLSTNKAVVSLSNGVSVLTSKVLDLKNYINNRLLPIVNQQSCRISNIETVIEFQQMNSRLLEITREFSVNAGVTTPLSTYMLTNSELLSLINDMPITNDQKKLMSSNVQIVRQQSYSIMSIIKEEVLAYVVQLPIYGVIDTPCWKLHTSPLCTTNIKEGSNICLTRTDRGWYCDNAGSVSFFPQADTCKVQSNRVFCDTMNSLTLPSEVSLCNTDIFNSKYDCKIMTSKTDISSSVITSLGAIVSCYGKTKCTASNKNRGIIKTFSNGCDYVSNKGVDTVSVGNTLYYVNKLEGKNLYVKGEPIINYYDPLVFPSDEFDASISQVNEKINQSLAFIRRSDELLHNVNTGKSTTNIMITTIIIVIIVVLLSLIAIGLLLYCKAKNTPVTLSKDQLSGINNIAFSK

SEQ ID NO: 3 - protein, 51 aa, synthetic construct
TPATNNRARKELPRFMNYTLNNAKKTNVTLSKKRKKKFLGFLLGVGSAIAS

SEQ ID NO: 4 - protein, 48 aa, synthetic construct
TPATNNRARQELPRFMNYTLNNAKKTNVTLSKKRFLGFLLGVGSAIAS

SEQ ID NO: 5 - protein, 51 aa, synthetic construct
TPATNNQAQNELPQFMNYTLNNANNTNVTLSQNQNQNFLGFLLGVGSAIAS

SEQ ID NO: 6 - protein, 51 aa, synthetic construct
TPATNNQAQNELPRFMNYTLNNAKKTNVTLSQNQNQNFLGFLLGVGSAIAS

SEQ ID NO: 7 - protein, 30 aa, synthetic construct
TPATNNQAQNQNQNQNFLGFLLGVGSAIAS

SEQ ID NO: 8 - protein, 28 aa, synthetic construct
TPATNNQAQNQNQNFLGFLLGVGSAIAS

SEQ ID NO: 9 - protein, 28 aa, synthetic construct
TPATNNRARQQQQRFLGFLLGVGSAIAS

SEQ ID NO: 10 - protein, 51 aa, synthetic construct
TPATNNRARRELPQFMNYTLNNAQQTNVTLSQNQNQNFLGFLLGVGSAIAS

SEQ ID NO: 11 - protein, 51 aa, synthetic construct
TPATNNQAQNELPQFMNYTLNNAQQTNVTLSKKRKRRFLGFLLGVGSAIAS

SEQ ID NO: 12 - protein, 42 aa, synthetic construct
TPATNNRARRELPRFMNYTLNNAKKTNVTLSKKRKRRSAIAS

SEQ ID NO: 13 - protein, 51 aa, synthetic construct
TPATNNIEGRELPRFMNYTLNNAKKTNVTLSKKIEGRFLGFLLGVGSAIAS

SEQ ID NO: 14 - protein, 64 aa, synthetic construct
PLVFPSDEFDASISQVNEKINQSLAFIRKSDELLHNVNDKIEEILSKIYHIENEIARIKKLIGE

SEQ ID NO: 15 - protein, 60 aa, synthetic construct
PLVFPSDEFDASISQVNEKINQSLAFIRKSDELLHNVNEKFHQIEKEFSEVEGRIQDLEK

SEQ ID NO: 16 - protein, 38 aa, synthetic construct
PLVFPSDEFDASISQINEKINQILAFIRKIDELLHNIN

SEQ ID NO: 17 - protein, 67 aa, synthetic construct
PLVFPSDEFDASISQVNEKINQSLAFIRKSDELLHNVNGSGYIPEAPRDGQAYVRKDGEWVLLSTFL

SEQ ID NO: 18 - protein, 73 aa, synthetic construct
PLVFPSDEFDASISQVNEKINQSLAFIRKSDELLHNVNNKNDDKGSGYIPEAPRDGQAYVRKDGEWVLLSTFL

SEQ ID NO: 19 - protein, 29 aa, unidentified
GSGYIPEAPRDGQAYVRKDGEWVLLSTFL

SEQ ID NO: 20 - protein, 31 aa, synthetic construct
KQIEDKIEEILSKIYHIENEIARIKKLIGEA

SEQ ID NO: 21 - protein, 574 aa, Human respiratory syncytial virus
MELLILKANAITTILTAVTFCFASGQNITEEFYQSTCSAVSKGYLSALRTGWYTSVITIELSNIKENKCNGTDAKVKLIKQELDKYKNAVTELQLLMQSTPATNNRARRELPRFMNYTLNNAKKTNVTLSKKRKRRFLGFLLGVGSAIASGVAVSKVLHLEGEVNKIKSALLSTNKAVVSLSNGVSVLTSKVLDLKNYIDKQLLPIVNKQSCSISNIETVIEFQQKNNRLLEITREFSVNAGVTTPVSTYMLTNSELLSLINDMPITNDQKKLMSNNVQIVRQQSYSIMSIIKEEVLAYVVQLPLYGVIDTPCWKLHTSPLCTTNTKEGSNICLTRTDRGWYCDNAGSVSFFPQAETCKVQSNRVFCDTMNSLTLPSEVNLCNVDIFNPKYDCKIMTSKTDVSSSVITSLGAIVSCYGKTKCTASNKNRGIIKTFSNGCDYVSNKGVDTVSVGNTLYYVNKQEGKSLYVKGEPIINFYDPLVFPSDEFDASISQVNEKINQSLAFIRKSDELLHNVNAGKSTTNIMITTIIIVIIVILLSLIAVGLLLYCKARSTPVTLSKDQLSGINNIAFSN

SEQ ID NO: 22 - DNA, 1727 bp, Human respiratory syncytial virus
  source 1..1727: mol_type = other DNA
atggaactgctgatcctgaaggccaacgccatcaccaccatcctgaccgccgtgaccttctgcttcgccagcggccagaacatcaccgaggaattctaccagagcacctgcagcgccgtgagcaagggctacctgagcgccctgcggaccggctggtacaccagcgtgatcaccatcgagctgtccaacatcaaagaaaacaagtgcaacggcaccgacgccaaggtgaaactgatcaagcaggaactggacaagtacaagaacgccgtgaccgagctgcagctgctgatgcagagcacccccgccaccaacaaccgggccagaagagagctgccccggttcatgaactacaccctgaacaacgccaagaaaaccaacgtgaccctgagcaagaagcggaagcggcggttcctgggcttcctgctgggcgtgggcagcgccatcgccagcggggtggccgtgtccaaggtgctgcacctggaaggcgaggtgaacaagatcaagtccgccctgctgtccaccaacaaggccgtggtgtccctgagcaacggcgtgagcgtgctgaccagcaaggtgctggatctgaagaactacatcgacaagcagctgctgcccatcgtgaacaagcagagctgcagcatcagcaacatcgagaccgtgatcgagttccagcagaagaacaaccggctgctggaaatcacccgggagttcagcgtgaacgccggcgtgaccacccccgtgagcacctacatgctgaccaacagcgagctgctgtccctgatcaatgacatgcccatcaccaacgaccagaaaaagctgatgagcaacaacgtgcagatcgtgcggcagcagagctactccatcatgagcatcatcaaagaagaggtgctggcctacgtggtgcagctgcccctgtacggcgtgatcgacaccccctgctggaagctgcacaccagccccctgtgcaccaccaacaccaaagagggcagcaacatctgcctgacccggaccgaccggggctggtactgcgacaacgccggcagcgtgagcttcttcccccaagccgagacctgcaaggtgcagagcaaccgggtgttctgcgacaccatgaacagcctgaccctgccctccgaggtgaacctgtgcaacgtggacatcttcaaccccaagtacgactgcaagatcatgacctccaagaccgacgtgagcagctccgtgatcacctccctgggcgccatcgtgagctgctacggcaagaccaagtgcaccgccagcaacaagaaccggggcatcatcaagaccttcagcaacggctgcgactacgtgagcaacaagggcgtggacaccgtgagcgtgggcaacacactgtactacgtgaataagcaggaaggcaagagcctgtacgtgaagggcgagcccatcatcaacttctacgaccccctggtgttccccagcgacgagttcgacgccagcatcagccaggtcaacgagaagatcaaccagagcctggccttcatccggaagagcgacgagctgctgcacaatgtgaatgccggcaagagcaccaccaatatcatgatcaccacaatcatcatcgtgatcattgtgatcctgctgtctctgattgccgtgggcctgctgctgtactgcaaggcccgcagcacccctgtgaccctgtccaaggaccagctgtccggcatcaacaatatcgccttctccaactgaag

SEQ ID NO: 23 - protein, 588 aa, synthetic construct
MELLILKANAITTILTAVTFCFASGQNITEEFYQSTCSAVSKGYLSALRTGWYTSVITIELSNIKENKCNGTDAKVKLIKQELDKYKNAVTELQLLMQSTPATNNRARRELPRFMNYTLNNAKKTNVTLSKKRKRRFLGFLLGVGSAIASGVAVSKVLHLEGEVNKIKSALLSTNKAVVSLSNGVSVLTSKVLDLKNYIDKQLLPIVNKQSCSISNIETVIEFQQKNNRLLEITREFSVNAGVTTPVSTYMLTNSELLSLINDMPITNDQKKLMSNNVQIVRQQSYSIMSIIKEEVLAYVVQLPLYGVIDTPCWKLHTSPLCTTNTKEGSNICLTRTDRGWYCDNAGSVSFFPQAETCKVQSNRVFCDTMNSLTLPSEVNLCNVDIFNPKYDCKIMTSKTDVSSSVITSLGAIVSCYGKTKCTASNKNRGIIKTFSNGCDYVSNKGVDTVSVGNTLYYVNKQEGKSLYVKGEPIINFYDPLVFPSDEFDASISQVNEKINQSLAFIRKSDELLHNVNAGKSTTNIMITTIIIVIIVILLSLIAVGLLLYCKARSTPVTLSKDQLSGINNIAFSNSGGSAGSGHHHHHH

SEQ ID NO: 24 - DNA, 1769 bp, synthetic construct
  source 1..1769: mol_type = other DNA
atggaactgctgatcctgaaggccaacgccatcaccaccatcctgaccgccgtgaccttctgcttcgccagcggccagaacatcaccgaggaattctaccagagcacctgcagcgccgtgagcaagggctacctgagcgccctgcggaccggctggtacaccagcgtgatcaccatcgagctgtccaacatcaaagaaaacaagtgcaacggcaccgacgccaaggtgaaactgatcaagcaggaactggacaagtacaagaacgccgtgaccgagctgcagctgctgatgcagagcacccccgccaccaacaaccgggccagaagagagctgccccggttcatgaactacaccctgaacaacgccaagaaaaccaacgtgaccctgagcaagaagcggaagcggcggttcctgggcttcctgctgggcgtgggcagcgccatcgccagcggggtggccgtgtccaaggtgctgcacctggaaggcgaggtgaacaagatcaagtccgccctgctgtccaccaacaaggccgtggtgtccctgagcaacggcgtgagcgtgctgaccagcaaggtgctggatctgaagaactacatcgacaagcagctgctgcccatcgtgaacaagcagagctgcagcatcagcaacatcgagaccgtgatcgagttccagcagaagaacaaccggctgctggaaatcacccgggagttcagcgtgaacgccggcgtgaccacccccgtgagcacctacatgctgaccaacagcgagctgctgtccctgatcaatgacatgcccatcaccaacgaccagaaaaagctgatgagcaacaacgtgcagatcgtgcggcagcagagctactccatcatgagcatcatcaaagaagaggtgctggcctacgtggtgcagctgcccctgtacggcgtgatcgacaccccctgctggaagctgcacaccagccccctgtgcaccaccaacaccaaagagggcagcaacatctgcctgacccggaccgaccggggctggtactgcgacaacgccggcagcgtgagcttcttcccccaagccgagacctgcaaggtgcagagcaaccgggtgttctgcgacaccatgaacagcctgaccctgccctccgaggtgaacctgtgcaacgtggacatcttcaaccccaagtacgactgcaagatcatgacctccaagaccgacgtgagcagctccgtgatcacctccctgggcgccatcgtgagctgctacggcaagaccaagtgcaccgccagcaacaagaaccggggcatcatcaagaccttcagcaacggctgcgactacgtgagcaacaagggcgtggacaccgtgagcgtgggcaacacactgtactacgtgaataagcaggaaggcaagagcctgtacgtgaagggcgagcccatcatcaacttctacgaccccctggtgttccccagcgacgagttcgacgccagcatcagccaggtcaacgagaagatcaaccagagcctggccttcatccggaagagcgacgagctgctgcacaatgtgaatgccggcaagagcaccaccaatatcatgatcaccacaatcatcatcgtgatcattgtgatcctgctgtctctgattgccgtgggcctgctgctgtactgcaaggcccgcagcacccctgtgaccctgtccaaggaccagctgtccggcatcaacaatatcgccttctccaacagcggcggcagcgccggctctggccaccaccaccatcaccactgaag

SEQ ID NO: 25 - protein, 624 aa, synthetic construct
MELLILKANAITTILTAVTFCFASGQNITEEFYQSTCSAVSKGYLSALRTGWYTSVITIELSNIKENKCNGTDAKVKLIKQELDKYKNAVTELQLLMQSTPATNNRARRELPRFMNYTLNNAKKTNVTLSKKRKRRFLGFLLGVGSAIASGVAVSKVLHLEGEVNKIKSALLSTNKAVVSLSNGVSVLTSKVLDLKNYIDKQLLPIVNKQSCSISNIETVIEFQQKNNRLLEITREFSVNAGVTTPVSTYMLTNSELLSLINDMPITNDQKKLMSNNVQIVRQQSYSIMSIIKEEVLAYVVQLPLYGVIDTPCWKLHTSPLCTTNTKEGSNICLTRTDRGWYCDNAGSVSFFPQAETCKVQSNRVFCDTMNSLTLPSEVNLCNVDIFNPKYDCKIMTSKTDVSSSVITSLGAIVSCYGKTKCTASNKNRGIIKTFSNGCDYVSNKGVDTVSVGNTLYYVNKQEGKSLYVKGEPIINFYDPLVFPSDEFDASISQVNEKINQSLAFIRKSDELLHNVNAGKSTTNIMITTIIIVIIVILLSLIAVGLLLYCKARSTPVTLSKDQLSGINNIAFSNGSSGRMKQIEDKIEEILSKIYHIENEIARIKKLIGESGGSAGSGHHHHHH

SEQ ID NO: 26 - DNA, 1877 bp, synthetic construct
  source 1..1877: mol_type = other DNA
atggaactgctgatcctgaaggccaacgccatcaccaccatcctgaccgccgtgaccttctgcttcgccagcggccagaacatcaccgaggaattctaccagagcacctgcagcgccgtgagcaagggctacctgagcgccctgcggaccggctggtacaccagcgtgatcaccatcgagctgtccaacatcaaagaaaacaagtgcaacggcaccgacgccaaggtgaaactgatcaagcaggaactggacaagtacaagaacgccgtgaccgagctgcagctgctgatgcagagcacccccgccaccaacaaccgggccagaagagagctgccccggttcatgaactacaccctgaacaacgccaagaaaaccaacgtgaccctgagcaagaagcggaagcggcggttcctgggcttcctgctgggcgtgggcagcgccatcgccagcggggtggccgtgtccaaggtgctgcacctggaaggcgaggtgaacaagatcaagtccgccctgctgtccaccaacaaggccgtggtgtccctgagcaacggcgtgagcgtgctgaccagcaaggtgctggatctgaagaactacatcgacaagcagctgctgcccatcgtgaacaagcagagctgcagcatcagcaacatcgagaccgtgatcgagttccagcagaagaacaaccggctgctggaaatcacccgggagttcagcgtgaacgccggcgtgaccacccccgtgagcacctacatgctgaccaacagcgagctgctgtccctgatcaatgacatgcccatcaccaacgaccagaaaaagctgatgagcaacaacgtgcagatcgtgcggcagcagagctactccatcatgagcatcatcaaagaagaggtgctggcctacgtggtgcagctgcccctgtacggcgtgatcgacaccccctgctggaagctgcacaccagccccctgtgcaccaccaacaccaaagagggcagcaacatctgcctgacccggaccgaccggggctggtactgcgacaacgccggcagcgtgagcttcttcccccaagccgagacctgcaaggtgcagagcaaccgggtgttctgcgacaccatgaacagcctgaccctgccctccgaggtgaacctgtgcaacgtggacatcttcaaccccaagtacgactgcaagatcatgacctccaagaccgacgtgagcagctccgtgatcacctccctgggcgccatcgtgagctgctacggcaagaccaagtgcaccgccagcaacaagaaccggggcatcatcaagaccttcagcaacggctgcgactacgtgagcaacaagggcgtggacaccgtgagcgtgggcaacacactgtactacgtgaataagcaggaaggcaagagcctgtacgtgaagggcgagcccatcatcaacttctacgaccccctggtgttccccagcgacgagttcgacgccagcatcagccaggtcaacgagaagatcaaccagagcctggccttcatccggaagagcgacgagctgctgcacaatgtgaatgccggcaagagcaccaccaatatcatgatcaccacaatcatcatcgtgatcattgtgatcctgctgtctctgattgccgtgggcctgctgctgtactgcaaggcccgcagcacccctgtgaccctgtccaaggaccagctgtccggcatcaacaatatcgccttctccaacggcagcagcggccggatgaagcagatcgaggacaagatcgaggaaatcctgagcaagatctaccacatcgagaacgagatcgcccggatcaagaagctgatcggcgaaagcggcggctctgccggaagcggccaccaccaccatcaccactgaag

SEQ ID NO: 27 - protein, 626 aa, synthetic construct
MELLILKANAITTILTAVTFCFASGQNITEEFYQSTCSAVSKGYLSALRTGWYTSVITIELSNIKENKCNGTDAKVKLIKQELDKYKNAVTELQLLMQSTPATNNRARRELPRFMNYTLNNAKKTNVTLSKKRKRRFLGFLLGVGSAIASGVAVSKVLHLEGEVNKIKSALLSTNKAVVSLSNGVSVLTSKVLDLKNYIDKQLLPIVNKQSCSISNIETVIEFQQKNNRLLEITREFSVNAGVTTPVSTYMLTNSELLSLINDMPITNDQKKLMSNNVQIVRQQSYSIMSIIKEEVLAYVVQLPLYGVIDTPCWKLHTSPLCTTNTKEGSNICLTRTDRGWYCDNAGSVSFFPQAETCKVQSNRVFCDTMNSLTLPSEVNLCNVDIFNPKYDCKIMTSKTDVSSSVITSLGAIVSCYGKTKCTASNKNRGIIKTFSNGCDYVSNKGVDTVSVGNTLYYVNKQEGKSLYVKGEPIINFYDPLVFPSDEFDASISQVNEKINQSLAFIRKSDELLHNVNAGKSTTNIMITTIIIVIIVILLSLIAVGLLLYCKARSTPVTLSKDQLSGINNIAFSNGSSGSGRMKQIEDKIEEILSKIYHIENEIARIKKLIGESGGSAGSGHHHHHH

SEQ ID NO: 28 - DNA, 1883 bp, synthetic construct
  source 1..1883: mol_type = other DNA
atggaactgctgatcctgaaggccaacgccatcaccaccatcctgaccgccgtgaccttctgcttcgccagcggccagaacatcaccgaggaattctaccagagcacctgcagcgccgtgagcaagggctacctgagcgccctgcggaccggctggtacaccagcgtgatcaccatcgagctgtccaacatcaaagaaaacaagtgcaacggcaccgacgccaaggtgaaactgatcaagcaggaactggacaagtacaagaacgccgtgaccgagctgcagctgctgatgcagagcacccccgccaccaacaaccgggccagaagagagctgccccggttcatgaactacaccctgaacaacgccaagaaaaccaacgtgaccctgagcaagaagcggaagcggcggttcctgggcttcctgctgggcgtgggcagcgccatcgccagcggggtggccgtgtccaaggtgctgcacctggaaggcgaggtgaacaagatcaagtccgccctgctgtccaccaacaaggccgtggtgtccctgagcaacggcgtgagcgtgctgaccagcaaggtgctggatctgaagaactacatcgacaagcagctgctgcccatcgtgaacaagcagagctgcagcatcagcaacatcgagaccgtgatcgagttccagcagaagaacaaccggctgctggaaatcacccgggagttcagcgtgaacgccggcgtgaccacccccgtgagcacctacatgctgaccaacagcgagctgctgtccctgatcaatgacatgcccatcaccaacgaccagaaaaagctgatgagcaacaacgtgcagatcgtgcggcagcagagctactccatcatgagcatcatcaaagaagaggtgctggcctacgtggtgcagctgcccctgtacggcgtgatcgacaccccctgctggaagctgcacaccagccccctgtgcaccaccaacaccaaagagggcagcaacatctgcctgacccggaccgaccggggctggtactgcgacaacgccggcagcgtgagcttcttcccccaagccgagacctgcaaggtgcagagcaaccgggtgttctgcgacaccatgaacagcctgaccctgccctccgaggtgaacctgtgcaacgtggacatcttcaaccccaagtacgactgcaagatcatgacctccaagaccgacgtgagcagctccgtgatcacctccctgggcgccatcgtgagctgctacggcaagaccaagtgcaccgccagcaacaagaaccggggcatcatcaagaccttcagcaacggctgcgactacgtgagcaacaagggcgtggacaccgtgagcgtgggcaacacactgtactacgtgaataagcaggaaggcaagagcctgtacgtgaagggcgagcccatcatcaacttctacgaccccctggtgttccccagcgacgagttcgacgccagcatcagccaggtcaacgagaagatcaaccagagcctggccttcatccggaagagcgacgagctgctgcacaatgtgaatgccggcaagagcaccaccaatatcatgatcaccacaatcatcatcgtgatcattgtgatcctgctgtctctgattgccgtgggcctgctgctgtactgcaaggcccgcagcacccctgtgaccctgtccaaggaccagctgtccggcatcaacaatatcgccttctccaacggcagcagcggcagcggccggatgaagcagatcgaggacaagatcgaggaaatcctgagcaagatctaccacatcgagaacgagatcgcccggatcaagaagctgatcggcgaaagcggcggctctgccggaagcggccaccaccaccatcaccactgaag

SEQ ID NO: 29 - protein, 531 aa, synthetic construct
MELLILKANAITTILTAVTFCFASGQNITEEFYQSTCSAVSKGYLSALRTGWYTSVITIELSNIKENKCNGTDAKVKLIKQELDKYKNAVTELQLLMQSTPATNNRARRELPRFMNYTLNNAKKTNVTLSKKRKRRFLGFLLGVGSAIASGVAVSKVLHLEGEVNKIKSALLSTNKAVVSLSNGVSVLTSKVLDLKNYIDKQLLPIVNKQSCSISNIETVIEFQQKNNRLLEITREFSVNAGVTTPVSTYMLTNSELLSLINDMPITNDQKKLMSNNVQIVRQQSYSIMSIIKEEVLAYVVQLPLYGVIDTPCWKLHTSPLCTTNTKEGSNICLTRTDRGWYCDNAGSVSFFPQAETCKVQSNRVFCDTMNSLTLPSEVNLCNVDIFNPKYDCKIMTSKTDVSSSVITSLGAIVSCYGKTKCTASNKNRGIIKTFSNGCDYVSNKGVDTVSVGNTLYYVNKQEGKSLYVKGEPIINFYDPLVFPSDEFDASISQVNEKINQSLAFIRKSDELLHNVNSGGSAGSGHHHHHH

SEQ ID NO: 30 - DNA, 1598 bp, synthetic construct
  source 1..1598: mol_type = other DNA
atggaactgctgatcctgaaggccaacgccatcaccaccatcctgaccgccgtgaccttctgcttcgccagcggccagaacatcaccgaggaattctaccagagcacctgcagcgccgtgagcaagggctacctgagcgccctgcggaccggctggtacaccagcgtgatcaccatcgagctgtccaacatcaaagaaaacaagtgcaacggcaccgacgccaaggtgaaactgatcaagcaggaactggacaagtacaagaacgccgtgaccgagctgcagctgctgatgcagagcacccccgccaccaacaaccgggccagaagagagctgccccggttcatgaactacaccctgaacaacgccaagaaaaccaacgtgaccctgagcaagaagcggaagcggcggttcctgggcttcctgctgggcgtgggcagcgccatcgccagcggggtggccgtgtccaaggtgctgcacctggaaggcgaggtgaacaagatcaagtccgccctgctgtccaccaacaaggccgtggtgtccctgagcaacggcgtgagcgtgctgaccagcaaggtgctggatctgaagaactacatcgacaagcagctgctgcccatcgtgaacaagcagagctgcagcatcagcaacatcgagaccgtgatcgagttccagcagaagaacaaccggctgctggaaatcacccgggagttcagcgtgaacgccggcgtgaccacccccgtgagcacctacatgctgaccaacagcgagctgctgtccctgatcaatgacatgcccatcaccaacgaccagaaaaagctgatgagcaacaacgtgcagatcgtgcggcagcagagctactccatcatgagcatcatcaaagaagaggtgctggcctacgtggtgcagctgcccctgtacggcgtgatcgacaccccctgctggaagctgcacaccagccccctgtgcaccaccaacaccaaagagggcagcaacatctgcctgacccggaccgaccggggctggtactgcgacaacgccggcagcgtgagcttcttcccccaagccgagacctgcaaggtgcagagcaaccgggtgttctgcgacaccatgaacagcctgaccctgccctccgaggtgaacctgtgcaacgtggacatcttcaaccccaagtacgactgcaagatcatgacctccaagaccgacgtgagcagctccgtgatcacctccctgggcgccatcgtgagctgctacggcaagaccaagtgcaccgccagcaacaagaaccggggcatcatcaagaccttcagcaacggctgcgactacgtgagcaacaagggcgtggacaccgtgagcgtgggcaacacactgtactacgtgaataagcaggaaggcaagagcctgtacgtgaagggcgagcccatcatcaacttctacgaccccctggtgttccccagcgacgagttcgacgccagcatcagccaggtcaacgagaagatcaaccagagcctggccttcatccggaagagcgacgagctgctgcacaatgtgaatagcggcggcagcgccggctctggccaccaccaccatcaccactgaag

SEQ ID NO: 31 - protein, 557 aa, synthetic construct
MELLILKANAITTILTAVTFCFASGQNITEEFYQSTCSAVSKGYLSALRTGWYTSVITIELSNIKENKCNGTDAKVKLIKQELDKYKNAVTELQLLMQSTPATNNRARRELPRFMNYTLNNAKKTNVTLSKKRKRRFLGFLLGVGSAIASGVAVSKVLHLEGEVNKIKSALLSTNKAVVSLSNGVSVLTSKVLDLKNYIDKQLLPIVNKQSCSISNIETVIEFQQKNNRLLEITREFSVNAGVTTPVSTYMLTNSELLSLINDMPITNDQKKLMSNNVQIVRQQSYSIMSIIKEEVLAYVVQLPLYGVIDTPCWKLHTSPLCTTNTKEGSNICLTRTDRGWYCDNAGSVSFFPQAETCKVQSNRVFCDTMNSLTLPSEVNLCNVDIFNPKYDCKIMTSKTDVSSSVITSLGAIVSCYGKTKCTASNKNRGIIKTFSNGCDYVSNKGVDTVSVGNTLYYVNKQEGKSLYVKGEPIINFYDPLVFPSDEFDASISQVNEKINQSLAFIRKSDELLHNVNDKIEEILSKIYHIENEIARIKKLIGESGGSAGSGHHHHHH

SEQ ID NO: 32 - DNA, 1676 bp, synthetic construct
  source 1..1676: mol_type = other DNA
atggaactgctgatcctgaaggccaacgccatcaccaccatcctgaccgccgtgaccttctgcttcgccagcggccagaacatcaccgaggaattctaccagagcacctgcagcgccgtgagcaagggctacctgagcgccctgcggaccggctggtacaccagcgtgatcaccatcgagctgtccaacatcaaagaaaacaagtgcaacggcaccgacgccaaggtgaaactgatcaagcaggaactggacaagtacaagaacgccgtgaccgagctgcagctgctgatgcagagcacccccgccaccaacaaccgggccagaagagagctgccccggttcatgaactacaccctgaacaacgccaagaaaaccaacgtgaccctgagcaagaagcggaagcggcggttcctgggcttcctgctgggcgtgggcagcgccatcgccagcggggtggccgtgtccaaggtgctgcacctggaaggcgaggtgaacaagatcaagtccgccctgctgtccaccaacaaggccgtggtgtccctgagcaacggcgtgagcgtgctgaccagcaaggtgctggatctgaagaactacatcgacaagcagctgctgcccatcgtgaacaagcagagctgcagcatcagcaacatcgagaccgtgatcgagttccagcagaagaacaaccggctgctggaaatcacccgggagttcagcgtgaacgccggcgtgaccacccccgtgagcacctacatgctgaccaacagcgagctgctgtccctgatcaatgacatgcccatcaccaacgaccagaaaaagctgatgagcaacaacgtgcagatcgtgcggcagcagagctactccatcatgagcatcatcaaagaagaggtgctggcctacgtggtgcagctgcccctgtacggcgtgatcgacaccccctgctggaagctgcacaccagccccctgtgcaccaccaacaccaaagagggcagcaacatctgcctgacccggaccgaccggggctggtactgcgacaacgccggcagcgtgagcttcttcccccaagccgagacctgcaaggtgcagagcaaccgggtgttctgcgacaccatgaacagcctgaccctgccctccgaggtgaacctgtgcaacgtggacatcttcaaccccaagtacgactgcaagatcatgacctccaagaccgacgtgagcagctccgtgatcacctccctgggcgccatcgtgagctgctacggcaagaccaagtgcaccgccagcaacaagaaccggggcatcatcaagaccttcagcaacggctgcgactacgtgagcaacaagggcgtggacaccgtgagcgtgggcaacacactgtactacgtgaataagcaggaaggcaagagcctgtacgtgaagggcgagcccatcatcaacttctacgaccccctggtgttccccagcgacgagttcgacgccagcatcagccaggtcaacgagaagatcaaccagagcctggccttcatccggaagagcgacgagctgctgcacaatgtgaatgacaagatcgaggaaatcctgagcaagatctaccacatcgagaacgagatcgcccggatcaagaagctgatcggcgaaagcggcggctctgccggaagcggccaccaccaccatcaccactgaag

SEQ ID NO: 33 - protein, 615 aa, synthetic construct
MELLILKANAITTILTAVTFCFASGQNITEEFYQSTCSAVSKGYLSALRTGWYTSVITIELSNIKENKCNGTDAKVKLIKQELDKYKNAVTELQLLMQSTPATNNRARRELPRFMNYTLNNAKKTNVTLSKKRKRRFLGFLLGVGSAIASGVAVSKVLHLEGEVNKIKSALLSTNKAVVSLSNGVSVLTSKVLDLKNYIDKQLLPIVNKQSCSISNIETVIEFQQKNNRLLEITREFSVNAGVTTPVSTYMLTNSELLSLINDMPITNDQKKLMSNNVQIVRQQSYSIMSIIKEEVLAYVVQLPLYGVIDTPCWKLHTSPLCTTNTKEGSNICLTRTDRGWYCDNAGSVSFFPQAETCKVQSNRVFCDTMNSLTLPSEVNLCNVDIFNPKYDCKIMTSKTDVSSSVITSLGAIVSCYGKTKCTASNKNRGIIKTFSNGCDYVSNKGVDTVSVGNTLYYVNKQEGKSLYVKGEPIINFYDPLVFPSDEFDASISQVNEKINQSLAFIRKSDELLHNVNAGKSTTNIMITTIIIVIIVILLSLIAVGLLLYCKARSTPVTLSKDQLSGINNIAFSNGSSGNEKFHQIEKEFSEVEGRIQDLEKSGGSAGSGHHHHHH

SEQ ID NO: 34 - DNA, 1850 bp, synthetic construct
  source 1..1850: mol_type = other DNA
atggaactgctgatcctgaaggccaacgccatcaccaccatcctgaccgccgtgaccttctgcttcgccagcggccagaacatcaccgaggaattctaccagagcacctgcagcgccgtgagcaagggctacctgagcgccctgcggaccggctggtacaccagcgtgatcaccatcgagctgtccaacatcaaagaaaacaagtgcaacggcaccgacgccaaggtgaaactgatcaagcaggaactggacaagtacaagaacgccgtgaccgagctgcagctgctgatgcagagcacccccgccaccaacaaccgggccagaagagagctgccccggttcatgaactacaccctgaacaacgccaagaaaaccaacgtgaccctgagcaagaagcggaagcggcggttcctgggcttcctgctgggcgtgggcagcgccatcgccagcggggtggccgtgtccaaggtgctgcacctggaaggcgaggtgaacaagatcaagtccgccctgctgtccaccaacaaggccgtggtgtccctgagcaacggcgtgagcgtgctgaccagcaaggtgctggatctgaagaactacatcgacaagcagctgctgcccatcgtgaacaagcagagctgcagcatcagcaacatcgagaccgtgatcgagttccagcagaagaacaaccggctgctggaaatcacccgggagttcagcgtgaacgccggcgtgaccacccccgtgagcacctacatgctgaccaacagcgagctgctgtccctgatcaatgacatgcccatcaccaacgaccagaaaaagctgatgagcaacaacgtgcagatcgtgcggcagcagagctactccatcatgagcatcatcaaagaagaggtgctggcctacgtggtgcagctgcccctgtacggcgtgatcgacaccccctgctggaagctgcacaccagccccctgtgcaccaccaacaccaaagagggcagcaacatctgcctgacccggaccgaccggggctggtactgcgacaacgccggcagcgtgagcttcttcccccaagccgagacctgcaaggtgcagagcaaccgggtgttctgcgacaccatgaacagcctgaccctgccctccgaggtgaacctgtgcaacgtggacatcttcaaccccaagtacgactgcaagatcatgacctccaagaccgacgtgagcagctccgtgatcacctccctgggcgccatcgtgagctgctacggcaagaccaagtgcaccgccagcaacaagaaccggggcatcatcaagaccttcagcaacggctgcgactacgtgagcaacaagggcgtggacaccgtgagcgtgggcaacacactgtactacgtgaataagcaggaaggcaagagcctgtacgtgaagggcgagcccatcatcaacttctacgaccccctggtgttccccagcgacgagttcgacgccagcatcagccaggtcaacgagaagatcaaccagagcctggccttcatccggaagagcgacgagctgctgcacaatgtgaatgccggcaagagcaccaccaatatcatgatcaccacaatcatcatcgtgatcattgtgatcctgctgtctctgattgccgtgggcctgctgctgtactgcaaggcccgcagcacccctgtgaccctgtccaaggaccagctgtccggcatcaacaatatcgccttctccaacggcagcagcggcaatgagaagttccaccagatcgagaaagaattcagcgaggtggagggccggatccaggacctggaaaagagcggcggctctgccggaagcggccaccaccaccatcaccactgaag

SEQ ID NO: 35 - protein, 553 aa, synthetic construct
MELLILKANAITTILTAVTFCFASGQNITEEFYQSTCSAVSKGYLSALRTGWYTSVITIELSNIKENKCNGTDAKVKLIKQELDKYKNAVTELQLLMQSTPATNNRARRELPRFMNYTLNNAKKTNVTLSKKRKRRFLGFLLGVGSAIASGVAVSKVLHLEGEVNKIKSALLSTNKAVVSLSNGVSVLTSKVLDLKNYIDKQLLPIVNKQSCSISNIETVIEFQQKNNRLLEITREFSVNAGVTTPVSTYMLTNSELLSLINDMPITNDQKKLMSNNVQIVRQQSYSIMSIIKEEVLAYVVQLPLYGVIDTPCWKLHTSPLCTTNTKEGSNICLTRTDRGWYCDNAGSVSFFPQAETCKVQSNRVFCDTMNSLTLPSEVNLCNVDIFNPKYDCKIMTSKTDVSSSVITSLGAIVSCYGKTKCTASNKNRGIIKTFSNGCDYVSNKGVDTVSVGNTLYYVNKQEGKSLYVKGEPIINFYDPLVFPSDEFDASISQVNEKINQSLAFIRKSDELLHNVNEKFHQIEKEFSEVEGRIQDLEKSGGSAGSGHHHHHH

SEQ ID NO: 36 - DNA, 1664 bp, synthetic construct
  source 1..1664: mol_type = other DNA
atggaactgctgatcctgaaggccaacgccatcaccaccatcctgaccgccgtgaccttctgcttcgccagcggccagaacatcaccgaggaattctaccagagcacctgcagcgccgtgagcaagggctacctgagcgccctgcggaccggctggtacaccagcgtgatcaccatcgagctgtccaacatcaaagaaaacaagtgcaacggcaccgacgccaaggtgaaactgatcaagcaggaactggacaagtacaagaacgccgtgaccgagctgcagctgctgatgcagagcacccccgccaccaacaaccgggccagaagagagctgccccggttcatgaactacaccctgaacaacgccaagaaaaccaacgtgaccctgagcaagaagcggaagcggcggttcctgggcttcctgctgggcgtgggcagcgccatcgccagcggggtggccgtgtccaaggtgctgcacctggaaggcgaggtgaacaagatcaagtccgccctgctgtccaccaacaaggccgtggtgtccctgagcaacggcgtgagcgtgctgaccagcaaggtgctggatctgaagaactacatcgacaagcagctgctgcccatcgtgaacaagcagagctgcagcatcagcaacatcgagaccgtgatcgagttccagcagaagaacaaccggctgctggaaatcacccgggagttcagcgtgaacgccggcgtgaccacccccgtgagcacctacatgctgaccaacagcgagctgctgtccctgatcaatgacatgcccatcaccaacgaccagaaaaagctgatgagcaacaacgtgcagatcgtgcggcagcagagctactccatcatgagcatcatcaaagaagaggtgctggcctacgtggtgcagctgcccctgtacggcgtgatcgacaccccctgctggaagctgcacaccagccccctgtgcaccaccaacaccaaagagggcagcaacatctgcctgacccggaccgaccggggctggtactgcgacaacgccggcagcgtgagcttcttcccccaagccgagacctgcaaggtgcagagcaaccgggtgttctgcgacaccatgaacagcctgaccctgccctccgaggtgaacctgtgcaacgtggacatcttcaaccccaagtacgactgcaagatcatgacctccaagaccgacgtgagcagctccgtgatcacctccctgggcgccatcgtgagctgctacggcaagaccaagtgcaccgccagcaacaagaaccggggcatcatcaagaccttcagcaacggctgcgactacgtgagcaacaagggcgtggacaccgtgagcgtgggcaacacactgtactacgtgaataagcaggaaggcaagagcctgtacgtgaagggcgagcccatcatcaacttctacgaccccctggtgttccccagcgacgagttcgacgccagcatcagccaggtcaacgagaagatcaaccagagcctggccttcatccggaagagcgacgagctgctgcacaatgtgaatgagaagttccaccagatcgagaaagaattcagcgaggtggagggccggatccaggacctggaaaagagcggcggctctgccggaagcggccaccaccaccatcaccactgaag

SEQ ID NO: 37 - protein, 534 aa, synthetic construct
MELLILKANAITTILTAVTFCFASGQNITEEFYQSTCSAVSKGYLSALRTGWYTSVITIELSNIKENKCNGTDAKVKLIKQELDKYKNAVTELQLLMQSTPATNNRARRELPRFMNYTLNNAKKTNVTLSKKRKRRFLGFLLGVGSAIASGVAVSKVLHLEGEVNKIKSALLSTNKAVVSLSNGVSVLTSKVLDLKNYIDKQLLPIVNKQSCSISNIETVIEFQQKNNRLLEITREFSVNAGVTTPVSTYMLTNSELLSLINDMPITNDQKKLMSNNVQIVRQQSYSIMSIIKEEVLAYVVQLPLYGVIDTPCWKLHTSPLCTTNTKEGSNICLTRTDRGWYCDNAGSVSFFPQAETCKVQSNRVFCDTMNSLTLPSEVNLCNVDIFNPKYDCKIMTSKTDVSSSVITSLGAIVSCYGKTKCTASNKNRGIIKTFSNGCDYVSNKGVDTVSVGNTLYYVNKQEGKSLYVKGEPNIMITTIIIVIIVILLSLIAVGLLLYCKARSTPVTLSKDQLSGINNIAFSNMGGSHHHHHH

SEQ ID NO: 38 - DNA, 1607 bp, synthetic construct
  source 1..1607: mol_type = other DNA
atggaactgctgatcctgaaggccaacgccatcaccaccatcctgaccgccgtgaccttctgcttcgccagcggccagaacatcaccgaggaattctaccagagcacctgcagcgccgtgagcaagggctacctgagcgccctgcggaccggctggtacaccagcgtgatcaccatcgagctgtccaacatcaaagaaaacaagtgcaacggcaccgacgccaaggtgaaactgatcaagcaggaactggacaagtacaagaacgccgtgaccgagctgcagctgctgatgcagagcacccccgccaccaacaaccgggccagaagagagctgccccggttcatgaactacaccctgaacaacgccaagaaaaccaacgtgaccctgagcaagaagcggaagcggcggttcctgggcttcctgctgggcgtgggcagcgccatcgccagcggggtggccgtgtccaaggtgctgcacctggaaggcgaggtgaacaagatcaagtccgccctgctgtccaccaacaaggccgtggtgtccctgagcaacggcgtgagcgtgctgaccagcaaggtgctggatctgaagaactacatcgacaagcagctgctgcccatcgtgaacaagcagagctgcagcatcagcaacatcgagaccgtgatcgagttccagcagaagaacaaccggctgctggaaatcacccgggagttcagcgtgaacgccggcgtgaccacccccgtgagcacctacatgctgaccaacagcgagctgctgtccctgatcaatgacatgcccatcaccaacgaccagaaaaagctgatgagcaacaacgtgcagatcgtgcggcagcagagctactccatcatgagcatcatcaaagaagaggtgctggcctacgtggtgcagctgcccctgtacggcgtgatcgacaccccctgctggaagctgcacaccagccccctgtgcaccaccaacaccaaagagggcagcaacatctgcctgacccggaccgaccggggctggtactgcgacaacgccggcagcgtgagcttcttcccccaagccgagacctgcaaggtgcagagcaaccgggtgttctgcgacaccatgaacagcctgaccctgccctccgaggtgaacctgtgcaacgtggacatcttcaaccccaagtacgactgcaagatcatgacctccaagaccgacgtgagcagctccgtgatcacctccctgggcgccatcgtgagctgctacggcaagaccaagtgcaccgccagcaacaagaaccggggcatcatcaagaccttcagcaacggctgcgactacgtgagcaacaagggcgtggacaccgtgagcgtgggcaacacactgtactacgtgaataagcaggaaggcaagagcctgtacgtgaagggcgagcccaatatcatgatcaccacaatcatcatcgtgatcattgtgatcctgctgtctctgattgccgtgggcctgctgctgtactgcaaggcccgcagcacccctgtgaccctgtccaaggaccagctgtccggcatcaacaatatcgccttctccaacatggggggttctcatcatcatcatcatcattgaag

SEQ ID NO: 39 - protein, 524 aa, synthetic construct
MELLILKANAITTILTAVTFCFASGQNITEEFYQSTCSAVSKGYLSALRTGWYTSVITIELSNIKENKCNGTDAKVKLIKQELDKYKNAVTELQLLMQSTPATNNRARRELPRFMNYTLNNAKKTNVTLSKKRKRRFLGFLLGVGSAIASGVAVSKVLHLEGEVNKIKSALLSTNKAVVSLSNGVSVLTSKVLDLKNYIDKQLLPIVNKQSCSISNIETVIEFQQKNNRLLEITREFSVNAGVTTPVSTYMLTNSELLSLINDMPITNDQKKLMSNNVQIVRQQSYSIMSIIKEEVLAYVVQLPLYGVIDTPCWKLHTSPLCTTNTKEGSNICLTRTDRGWYCDNAGSVSFFPQAETCKVQSNRVFCDTMNSLTLPSEVNLCNVDIFNPKYDCKIMTSKTDVSSSVITSLGAIVSCYGKTKCTASNKNRGIIKTFSNGCDYVSNKGVDTVSVGNTLYYVNKQEGKSLYVKGEPIINFYDPLVFPSDEFDASISQVNEKINQSLAFIRKSDELLHNVNAGKSTTN

SEQ ID NO: 40 - DNA, 1577 bp, synthetic construct
  source 1..1577: mol_type = other DNA
atggaactgctgatcctgaaggccaacgccatcaccaccatcctgaccgccgtgaccttctgcttcgccagcggccagaacatcaccgaggaattctaccagagcacctgcagcgccgtgagcaagggctacctgagcgccctgcggaccggctggtacaccagcgtgatcaccatcgagctgtccaacatcaaagaaaacaagtgcaacggcaccgacgccaaggtgaaactgatcaagcaggaactggacaagtacaagaacgccgtgaccgagctgcagctgctgatgcagagcacccccgccaccaacaaccgggccagaagagagctgccccggttcatgaactacaccctgaacaacgccaagaaaaccaacgtgaccctgagcaagaagcggaagcggcggttcctgggcttcctgctgggcgtgggcagcgccatcgccagcggggtggccgtgtccaaggtgctgcacctggaaggcgaggtgaacaagatcaagtccgccctgctgtccaccaacaaggccgtggtgtccctgagcaacggcgtgagcgtgctgaccagcaaggtgctggatctgaagaactacatcgacaagcagctgctgcccatcgtgaacaagcagagctgcagcatcagcaacatcgagaccgtgatcgagttccagcagaagaacaaccggctgctggaaatcacccgggagttcagcgtgaacgccggcgtgaccacccccgtgagcacctacatgctgaccaacagcgagctgctgtccctgatcaatgacatgcccatcaccaacgaccagaaaaagctgatgagcaacaacgtgcagatcgtgcggcagcagagctactccatcatgagcatcatcaaagaagaggtgctggcctacgtggtgcagctgcccctgtacggcgtgatcgacaccccctgctggaagctgcacaccagccccctgtgcaccaccaacaccaaagagggcagcaacatctgcctgacccggaccgaccggggctggtactgcgacaacgccggcagcgtgagcttcttcccccaagccgagacctgcaaggtgcagagcaaccgggtgttctgcgacaccatgaacagcctgaccctgccctccgaggtgaacctgtgcaacgtggacatcttcaaccccaagtacgactgcaagatcatgacctccaagaccgacgtgagcagctccgtgatcacctccctgggcgccatcgtgagctgctacggcaagaccaagtgcaccgccagcaacaagaaccggggcatcatcaagaccttcagcaacggctgcgactacgtgagcaacaagggcgtggacaccgtgagcgtgggcaacacactgtactacgtgaataagcaggaaggcaagagcctgtacgtgaagggcgagcccatcatcaacttctacgaccccctggtgttccccagcgacgagttcgacgccagcatcagccaggtcaacgagaagatcaaccagagcctggccttcatccggaagagcgacgagctgctgcacaatgtgaatgccggcaagagcaccaccaattgaag

SEQ ID NO: 41 - protein, 574 aa, Human respiratory syncytial virus; identical to SEQ ID NO: 21

SEQ ID NO: 42 - protein, 590 aa, synthetic construct
MELLILKANAITTILTAVTFCFASGQNITEEFYQSTCSAVSKGYLSALRTGWYTSVITIELSNIKENKCNGTDAKVKLIKQELDKYKNAVTELQLLMQSTPATNNRARRELPRFMNYTLNNAKKTNVTLSKKRKRRFLGFLLGVGSAIASGVAVSKVLHLEGEVNKIKSALLSTNKAVVSLSNGVSVLTSKVLDLKNYIDKQLLPIVNKQSCSISNIETVIEFQQKNNRLLEITREFSVNAGVTTPVSTYMLTNSELLSLINDMPITNDQKKLMSNNVQIVRQQSYSIMSIIKEEVLAYVVQLPLYGVIDTPCWKLHTSPLCTTNTKEGSNICLTRTDRGWYCDNAGSVSFFPQAETCKVQSNRVFCDTMNSLTLPSEVNLCNVDIFNPKYDCKIMTSKTDVSSSVITSLGAIVSCYGKTKCTASNKNRGIIKTFSNGCDYVSNKGVDTVSVGNTLYYVNKQEGKSLYVKGEPIINFYDPLVFPSDEFDASISQINEKINQILAFIRKIDELLHNINAGKSTTNGSGSGDDDDDKGSGSGIMITTIIIVIIVILLSLIAVGLLLYCKARSTPVTLSKDQLSGINNIAFSN

SEQ ID NO: 43 - protein, 588 aa, synthetic construct
MELLILKANAITTILTAVTFCFASGQNITEEFYQSTCSAVSKGYLSALRTGWYTSVITIELSNIKENKCNGTDAKVKLIKQELDKYKNAVTELQLLMQSTPATNNRARRELPRFMNYTLNNAKKTNVTLSKKRKRRFLGFLLGVGSAIASGVAVSKVLHLEGEVNKIKSALLSTNKAVVSLSNGVSVLTSKVLDLKNYIDKQLLPIVNKQSCSISNIETVIEFQQKNNRLLEITREFSVNAGVTTPVSTYMLTNSELLSLINDMPITNDQKKLMSNNVQIVRQQSYSIMSIIKEEVLAYVVQLPLYGVIDTPCWKLHTSPLCTTNTKEGSNICLTRTDRGWYCDNAGSVSFFPQAETCKVQSNRVFCDTMNSLTLPSEVNLCNVDIFNPKYDCKIMTSKTDVSSSVITSLGAIVSCYGKTKCTASNKNRGIIKTFSNGCDYVSNKGVDTVSVGNTLYYVNKQEGKSLYVKGEPIINFYDPLVFPSDEFDASISQINEKINQILAFIRKIDELLHNINAGKSTTNGSGSGLVPRGSGSGIMITTIIIVIIVILLSLIAVGLLLYCKARSTPVTLSKDQLSGINNIAFSN

SEQ ID NO: 44 - protein, 588 aa, synthetic construct
MELLILKANAITTILTAVTFCFASGQNITEEFYQSTCSAVSKGYLSALRTGWYTSVITIELSNIKENKCNGTDAKVKLIKQELDKYKNAVTELQLLMQSTPATNNRARRELPRFMNYTLNNAKKTNVTLSKKRKRRFLGFLLGVGSAIASGVAVSKVLHLEGEVNKIKSALLSTNKAVVSLSNGVSVLTSKVLDLKNYIDKQLLPIVNKQSCSISNIETVIEFQQKNNRLLEITREFSVNAGVTTPVSTYMLTNSELLSLINDMPITNDQKKLMSNNVQIVRQQSYSIMSIIKEEVLAYVVQLPLYGVIDTPCWKLHTSPLCTTNTKEGSNICLTRTDRGWYCDNAGSVSFFPQAETCKVQSNRVFCDTMNSLTLPSEVNLCNVDIFNPKYDCKIMTSKTDVSSSVITSLGAIVSCYGKTKCTASNKNRGIIKTFSNGCDYVSNKGVDTVSVGNTLYYVNKQEGKSLYVKGEPIINFYDPLVFPSDEFDASISQINEKINQILAFIRKIDELLHNINAGKSTTNGSGSGIEGRGSGSGIMITTIIIVIIVILLSLIAVGLLLYCKARSTPVTLSKDQLSGINNIAFSN

SEQ ID NO: 45 - protein, 537 aa, synthetic construct
MELLILKANAITTILTAVTFCFASGQNITEEFYQSTCSAVSKGYLSALRTGWYTSVITIELSNIKENKCNGTDAKVKLIKQELDKYKNAVTELQLLMQSTPATNNQAQNELPRFMNYTLNNAKKTNVTLSQNQNQNFLGFLLGVGSAIASGVAVSKVLHLEGEVNKIKSALLSTNKAVVSLSNGVSVLTSKVLDLKNYIDKQLLPIVNKQSCSISNIETVIEFQQKNNRLLEITREFSVNAGVTTPVSTYMLTNSELLSLINDMPITNDQKKLMSNNVQIVRQQSYSIMSIIKEEVLAYVVQLPLYGVIDTPCWKLHTSPLCTTNTKEGSNICLTRTDRGWYCDNAGSVSFFPQAETCKVQSNRVFCDTMNSLTLPSEVNLCNVDIFNPKYDCKIMTSKTDVSSSVITSLGAIVSCYGKTKCTASNKNRGIIKTFSNGCDYVSNKGVDTVSVGNTLYYVNKQEGKSLYVKGEPIINFYDPLVFPSDEFDASISQVNEKINQSLAFIRKSDELLHNVNAGKSTTNGGSAGSGHHHHHH

SEQ ID NO: 46 - protein, 537 aa, synthetic construct
MELLILKANAITTILTAVTFCFASGQNITEEFYQSTCSAVSKGYLSALRTGWYTSVITIELSNIKENKCNGTDAKVKLIKQELDKYKNAVTELQLLMQSTPATNNQAQNELPQFMNYTLNNANNTNVTLSQNQNQNFLGFLLGVGSAIASGVAVSKVLHLEGEVNKIKSALLSTNKAVVSLSNGVSVLTSKVLDLKNYIDKQLLPIVNKQSCSISNIETVIEFQQKNNRLLEITREFSVNAGVTTPVSTYMLTNSELLSLINDMPITNDQKKLMSNNVQIVRQQSYSIMSIIKEEVLAYVVQLPLYGVIDTPCWKLHTSPLCTTNTKEGSNICLTRTDRGWYCDNAGSVSFFPQAETCKVQSNRVFCDTMNSLTLPSEVNLCNVDIFNPKYDCKIMTSKTDVSSSVITSLGAIVSCYGKTKCTASNKNRGIIKTFSNGCDYVSNKGVDTVSVGNTLYYVNKQEGKSLYVKGEPIINFYDPLVFPSDEFDASISQVNEKINQSLAFIRKSDELLHNVNAGKSTTNGGSAGSGHHHHHH

SEQ ID NO: 47 - protein, 516 aa, synthetic construct
MELLILKANAITTILTAVTFCFASGQNITEEFYQSTCSAVSKGYLSALRTGWYTSVITIELSNIKENKCNGTDAKVKLIKQELDKYKNAVTELQLLMQSTPATNNQAQNQNQNQNFLGFLLGVGSAIASGVAVSKVLHLEGEVNKIKSALLSTNKAVVSLSNGVSVLTSKVLDLKNYIDKQLLPIVNKQSCSISNIETVIEFQQKNNRLLEITREFSVNAGVTTPVSTYMLTNSELLSLINDMPITNDQKKLMSNNVQIVRQQSYSIMSIIKEEVLAYVVQLPLYGVIDTPCWKLHTSPLCTTNTKEGSNICLTRTDRGWYCDNAGSVSFFPQAETCKVQSNRVFCDTMNSLTLPSEVNLCNVDIFNPKYDCKIMTSKTDVSSSVITSLGAIVSCYGKTKCTASNKNRGIIKTFSNGCDYVSNKGVDTVSVGNTLYYVNKQEGKSLYVKGEPIINFYDPLVFPSDEFDASISQVNEKINQSLAFIRKSDELLHNVNAGKSTTNGGSAGSGHHHHHH

SEQ ID NO: 48 - protein, 514 aa, synthetic construct
MELLILKANAITTILTAVTFCFASGQNITEEFYQSTCSAVSKGYLSALRTGWYTSVITIELSNIKENKCNGTDAKVKLIKQELDKYKNAVTELQLLMQSTPATNNQAQNQNQNFLGFLLGVGSAIASGVAVSKVLHLEGEVNKIKSALLSTNKAVVSLSNGVSVLTSKVLDLKNYIDKQLLPIVNKQSCSISNIETVIEFQQKNNRLLEITREFSVNAGVTTPVSTYMLTNSELLSLINDMPITNDQKKLMSNNVQIVRQQSYSIMSIIKEEVLAYVVQLPLYGVIDTPCWKLHTSPLCTTNTKEGSNICLTRTDRGWYCDNAGSVSFFPQAETCKVQSNRVFCDTMNSLTLPSEVNLCNVDIFNPKYDCKIMTSKTDVSSSVITSLGAIVSCYGKTKCTASNKNRGIIKTFSNGCDYVSNKGVDTVSVGNTLYYVNKQEGKSLYVKGEPIINFYDPLVFPSDEFDASISQVNEKINQSLAFIRKSDELLHNVNAGKSTTNGGSAGSGHHHHHH

SEQ ID NO: 49 - protein, 514 aa, synthetic construct
MELLILKANAITTILTAVTFCFASGQNITEEFYQSTCSAVSKGYLSALRTGWYTSVITIELSNIKENKCNGTDAKVKLIKQELDKYKNAVTELQLLMQSTPATNNRARQQQQRFLGFLLGVGSAIASGVAVSKVLHLEGEVNKIKSALLSTNKAVVSLSNGVSVLTSKVLDLKNYIDKQLLPIVNKQSCSISNIETVIEFQQKNNRLLEITREFSVNAGVTTPVSTYMLTNSELLSLINDMPITNDQKKLMSNNVQIVRQQSYSIMSIIKEEVLAYVVQLPLYGVIDTPCWKLHTSPLCTTNTKEGSNICLTRTDRGWYCDNAGSVSFFPQAETCKVQSNRVFCDTMNSLTLPSEVNLCNVDIFNPKYDCKIMTSKTDVSSSVITSLGAIVSCYGKTKCTASNKNRGIIKTFSNGCDYVSNKGVDTVSVGNTLYYVNKQEGKSLYVKGEPIINFYDPLVFPSDEFDASISQVNEKINQSLAFIRKSDELLHNVNAGKSTTNGGSAGSGHHHHHH

SEQ ID NO: 50 - protein, 537 aa, synthetic construct
MELLILKANAITTILTAVTFCFASGQNITEEFYQSTCSAVSKGYLSALRTGWYTSVITIELSNIKENKCNGTDAKVKLIKQELDKYKNAVTELQLLMQSTPATNNRARKELPRFMNYTLNNAKKTNVTLSKKRKKKFLGFLLGVGSAIASGVAVSKVLHLEGEVNKIKSALLSTNKAVVSLSNGVSVLTSKVLDLKNYIDKQLLPIVNKQSCSISNIETVIEFQQKNNRLLEITREFSVNAGVTTPVSTYMLTNSELLSLINDMPITNDQKKLMSNNVQIVRQQSYSIMSIIKEEVLAYVVQLPLYGVIDTPCWKLHTSPLCTTNTKEGSNICLTRTDRGWYCDNAGSVSFFPQAETCKVQSNRVFCDTMNSLTLPSEVNLCNVDIFNPKYDCKIMTSKTDVSSSVITSLGAIVSCYGKTKCTASNKNRGIIKTFSNGCDYVSNKGVDTVSVGNTLYYVNKQEGKSLYVKGEPIINFYDPLVFPSDEFDASISQVNEKINQSLAFIRKSDELLHNVNAGKSTTNGGSAGSGHHHHHH

SEQ ID NO: 51 - protein, 534 aa, synthetic construct
MELLILKANAITTILTAVTFCFASGQNITEEFYQSTCSAVSKGYLSALRTGWYTSVITIELSNIKENKCNGTDAKVKLIKQELDKYKNAVTELQLLMQSTPATNNRARQELPRFMNYTLNNAKKTNVTLSKKRFLGFLLGVGSAIASGVAVSKVLHLEGEVNKIKSALLSTNKAVVSLSNGVSVLTSKVLDLKNYIDKQLLPIVNKQSCSISNIETVIEFQQKNNRLLEITREFSVNAGVTTPVSTYMLTNSELLSLINDMPITNDQKKLMSNNVQIVRQQSYSIMSIIKEEVLAYVVQLPLYGVIDTPCWKLHTSPLCTTNTKEGSNICLTRTDRGWYCDNAGSVSFFPQAETCKVQSNRVFCDTMNSLTLPSEVNLCNVDIFNPKYDCKIMTSKTDVSSSVITSLGAIVSCYGKTKCTASNKNRGIIKTFSNGCDYVSNKGVDTVSVGNTLYYVNKQEGKSLYVKGEPIINFYDPLVFPSDEFDASISQVNEKINQSLAFIRKSDELLHNVNAGKSTTNGGSAGSGHHHHHH

SEQ ID NO: 52 - protein, 537 aa, synthetic construct
MELLILKANAITTILTAVTFCFASGQNITEEFYQSTCSAVSKGYLSALRTGWYTSVITIELSNIKENKCNGTDAKVKLIKQELDKYKNAVTELQLLMQSTPATNNIEGRELPRFMNYTLNNAKKTNVTLSKKIEGRFLGFLLGVGSAIASGVAVSKVLHLEGEVNKIKSALLSTNKAVVSLSNGVSVLTSKVLDLKNYIDKQLLPIVNKQSCSISNIETVIEFQQKNNRLLEITREFSVNAGVTTPVSTYMLTNSELLSLINDMPITNDQKKLMSNNVQIVRQQSYSIMSIIKEEVLAYVVQLPLYGVIDTPCWKLHTSPLCTTNTKEGSNICLTRTDRGWYCDNAGSVSFFPQAETCKVQSNRVFCDTMNSLTLPSEVNLCNVDIFNPKYDCKIMTSKTDVSSSVITSLGAIVSCYGKTKCTASNKNRGIIKTFSNGCDYVSNKGVDTVSVGNTLYYVNKQEGKSLYVKGEPIINFYDPLVFPSDEFDASISQVNEKINQSLAFIRKSDELLHNVNAGKSTTNGGSAGSGHHHHHH

SEQ ID NO: 53 - protein, 566 aa, synthetic construct
MELLILKANAITTILTAVTFCFASGQNITEEFYQSTCSAVSKGYLSALRTGWYTSVITIELSNIKENKCNGTDAKVKLIKQELDKYKNAVTELQLLMQSTPATNNRARRELPRFMNYTLNNAKKTNVTLSKKRKRRFLGFLLGVGSAIASGVAVSKVLHLEGEVNKIKSALLSTNKAVVSLSNGVSVLTSKVLDLKNYIDKQLLPIVNKQSCSISNIETVIEFQQKNNRLLEITREFSVNAGVTTPVSTYMLTNSELLSLINDMPITNDQKKLMSNNVQIVRQQSYSIMSIIKEEVLAYVVQLPLYGVIDTPCWKLHTSPLCTTNTKEGSNICLTRTDRGWYCDNAGSVSFFPQAETCKVQSNRVFCDTMNSLTLPSEVNLCNVDIFNPKYDCKIMTSKTDVSSSVITSLGAIVSCYGKTKCTASNKNRGIIKTFSNGCDYVSNKGVDTVSVGNTLYYVNKQEGKSLYVKGEPIINFYDPLVFPSDEFDASISQVNEKINQSLAFIRKSDELLHNVNAGKSTTNGSGYIPEAPRDGQAYVRKDGEWVLLSTFLGGSAGSGHHHHHH

SEQ ID NO: 54 - protein, 572 aa, synthetic construct
MELLILKANAITTILTAVTFCFASGQNITEEFYQSTCSAVSKGYLSALRTGWYTSVITIELSNIKENKCNGTDAKVKLIKQELDKYKNAVTELQLLMQSTPATNNRARRELPRFMNYTLNNAKKTNVTLSKKRKRRFLGFLLGVGSAIASGVAVSKVLHLEGEVNKIKSALLSTNKAVVSLSNGVSVLTSKVLDLKNYIDKQLLPIVNKQSCSISNIETVIEFQQKNNRLLEITREFSVNAGVTTPVSTYMLTNSELLSLINDMPITNDQKKLMSNNVQIVRQQSYSIMSIIKEEVLAYVVQLPLYGVIDTPCWKLHTSPLCTTNTKEGSNICLTRTDRGWYCDNAGSVSFFPQAETCKVQSNRVFCDTMNSLTLPSEVNLCNVDIFNPKYDCKIMTSKTDVSSSVITSLGAIVSCYGKTKCTASNKNRGIIKTFSNGCDYVSNKGVDTVSVGNTLYYVNKQEGKSLYVKGEPIINFYDPLVFPSDEFDASISQVNEKINQSLAFIRKSDELLHNVNAGKSTTNNKNDDKGSGYIPEAPRDGQAYVRKDGEWVLLSTFLGGSAGSGHHHHHH

SEQ ID NO: 55 - protein, 557 aa, synthetic construct; identical to SEQ ID NO: 31

SEQ ID NO: 56 - protein, 553 aa, synthetic construct; identical to SEQ ID NO: 35

SEQ ID NO: 57 - protein, 557 aa, synthetic construct
MELLILKANAITTILTAVTFCFASGQNITEEFYQSTCSAVSKGYLSALRTGWYTSVITIELSNIKENKCNGTDAKVKLIKQELDKYKNAVTELQLLMQSTPATNNQAQNELPQFMNYTLNNANNTNVTLSQNQNQNFLGFLLGVGSAIASGVAVSKVLHLEGEVNKIKSALLSTNKAVVSLSNGVSVLTSKVLDLKNYIDKQLLPIVNKQSCSISNIETVIEFQQKNNRLLEITREFSVNAGVTTPVSTYMLTNSELLSLINDMPITNDQKKLMSNNVQIVRQQSYSIMSIIKEEVLAYVVQLPLYGVIDTPCWKLHTSPLCTTNTKEGSNICLTRTDRGWYCDNAGSVSFFPQAETCKVQSNRVFCDTMNSLTLPSEVNLCNVDIFNPKYDCKIMTSKTDVSSSVITSLGAIVSCYGKTKCTASNKNRGIIKTFSNGCDYVSNKGVDTVSVGNTLYYVNKQEGKSLYVKGEPIINFYDPLVFPSDEFDASISQVNEKINQSLAFIRKSDELLHNVNDKIEEILSKIYHIENEIARIKKLIGESGGSAGSGHHHHHH

SEQ ID NO: 58 - protein, 536 aa, synthetic construct
MELLILKANAITTILTAVTFCFASGQNITEEFYQSTCSAVSKGYLSALRTGWYTSVITIELSNIKENKCNGTDAKVKLIKQELDKYKNAVTELQLLMQSTPATNNQAQNQNQNQNFLGFLLGVGSAIASGVAVSKVLHLEGEVNKIKSALLSTNKAVVSLSNGVSVLTSKVLDLKNYIDKQLLPIVNKQSCSISNIETVIEFQQKNNRLLEITREFSVNAGVTTPVSTYMLTNSELLSLINDMPITNDQKKLMSNNVQIVRQQSYSIMSIIKEEVLAYVVQLPLYGVIDTPCWKLHTSPLCTTNTKEGSNICLTRTDRGWYCDNAGSVSFFPQAETCKVQSNRVFCDTMNSLTLPSEVNLCNVDIFNPKYDCKIMTSKTDVSSSVITSLGAIVSCYGKTKCTASNKNRGIIKTFSNGCDYVSNKGVDTVSVGNTLYYVNKQEGKSLYVKGEPIINFYDPLVFPSDEFDASISQVNEKINQSLAFIRKSDELLHNVNDKIEEILSKIYHIENEIARIKKLIGESGGSAGSGHHHHHH

SEQ ID NO: 59 - protein, 534 aa, synthetic construct
MELLILKANAITTILTAVTFCFASGQNITEEFYQSTCSAVSKGYLSALRTGWYTSVITIELSNIKENKCNGTDAKVKLIKQELDKYKNAVTELQLLMQSTPATNNQAQNQNQNFLGFLLGVGSAIASGVAVSKVLHLEGEVNKIKSALLSTNKAVVSLSNGVSVLTSKVLDLKNYIDKQLLPIVNKQSCSISNIETVIEFQQKNNRLLEITREFSVNAGVTTPVSTYMLTNSELLSLINDMPITNDQKKLMSNNVQIVRQQSYSIMSIIKEEVLAYVVQLPLYGVIDTPCWKLHTSPLCTTNTKEGSNICLTRTDRGWYCDNAGSVSFFPQAETCKVQSNRVFCDTMNSLTLPSEVNLCNVDIFNPKYDCKIMTSKTDVSSSVITSLGAIVSCYGKTKCTASNKNRGIIKTFSNGCDYVSNKGVDTVSVGNTLYYVNKQEGKSLYVKGEPIINFYDPLVFPSDEFDASISQVNEKINQSLAFIRKSDELLHNVNDKIEEILSKIYHIENEIARIKKLIGESGGSAGSGHHHHHH

SEQ ID NO: 60 - protein, 534 aa, synthetic construct
MELLILKANAITTILTAVTFCFASGQNITEEFYQSTCSAVSKGYLSALRTGWYTSVITIELSNIKENKCNGTDAKVKLIKQELDKYKNAVTELQLLMQSTPATNNRARQQQQRFLGFLLGVGSAIASGVAVSKVLHLEGEVNKIKSALLSTNKAVVSLSNGVSVLTSKVLDLKNYIDKQLLPIVNKQSCSISNIETVIEFQQKNNRLLEITREFSVNAGVTTPVSTYMLTNSELLSLINDMPITNDQKKLMSNNVQIVRQQSYSIMSIIKEEVLAYVVQLPLYGVIDTPCWKLHTSPLCTTNTKEGSNICLTRTDRGWYCDNAGSVSFFPQAETCKVQSNRVFCDTMNSLTLPSEVNLCNVDIFNPKYDCKIMTSKTDVSSSVITSLGAIVSCYGKTKCTASNKNRGIIKTFSNGCDYVSNKGVDTVSVGNTLYYVNKQEGKSLYVKGEPIINFYDPLVFPSDEFDASISQVNEKINQSLAFIRKSDELLHNVNDKIEEILSKIYHIENEIARIKKLIGESGGSAGSGHHHHHH

SEQ ID NO: 61 - protein, 574 aa, synthetic construct
MELLILKANAITTILTAVTFCFASGQNITEEFYQSTCSAVSKGYLSALRTGWYTSVITIELSNIKENKCNGTDAKVKLIKQELDKYKNAVTELQLLMQSTPATNNQAQNELPQFMNYTLNNANNTNVTLSQNQNQNFLGFLLGVGSAIASGVAVSKVLHLEGEVNKIKSALLSTNKAVVSLSNGVSVLTSKVLDLKNYIDKQLLPIVNKQSCSISNIETVIEFQQKNNRLLEITREFSVNAGVTTPVSTYMLTNSELLSLINDMPITNDQKKLMSNNVQIVRQQSYSIMSIIKEEVLAYVVQLPLYGVIDTPCWKLHTSPLCTTNTKEGSNICLTRTDRGWYCDNAGSVSFFPQAETCKVQSNRVFCDTMNSLTLPSEVNLCNVDIFNPKYDCKIMTSKTDVSSSVITSLGAIVSCYGKTKCTASNKNRGIIKTFSNGCDYVSNKGVDTVSVGNTLYYVNKQEGKSLYVKGEPIINFYDPLVFPSDEFDASISQVNEKINQSLAFIRKSDELLHNVNAGKSTTNIMITTIIIVIIVILLSLIAVGLLLYCKARSTPVTLSKDQLSGINNIAFSN

SEQ ID NO: 62 - protein, 553 aa, synthetic construct
MELLILKANAITTILTAVTFCFASGQNITEEFYQSTCSAVSKGYLSALRTGWYTSVITIELSNIKENKCNGTDAKVKLIKQELDKYKNAVTELQLLMQSTPATNNQAQNQNQNQNFLGFLLGVGSAIASGVAVSKVLHLEGEVNKIKSALLSTNKAVVSLSNGVSVLTSKVLDLKNYIDKQLLPIVNKQSCSISNIETVIEFQQKNNRLLEITREFSVNAGVTTPVSTYMLTNSELLSLINDMPITNDQKKLMSNNVQIVRQQSYSIMSIIKEEVLAYVVQLPLYGVIDTPCWKLHTSPLCTTNTKEGSNICLTRTDRGWYCDNAGSVSFFPQAETCKVQSNRVFCDTMNSLTLPSEVNLCNVDIFNPKYDCKIMTSKTDVSSSVITSLGAIVSCYGKTKCTASNKNRGIIKTFSNGCDYVSNKGVDTVSVGNTLYYVNKQEGKSLYVKGEPIINFYDPLVFPSDEFDASISQVNEKINQSLAFIRKSDELLHNVNAGKSTTNIMITTIIIVIIVILLSLIAVGLLLYCKARSTPVTLSKDQLSGINNIAFSN

SEQ ID NO: 63 - protein, 551 aa, synthetic construct
MELLILKANAITTILTAVTFCFASGQNITEEFYQSTCSAVSKGYLSALRTGWYTSVITIELSNIKENKCNGTDAKVKLIKQELDKYKNAVTELQLLMQSTPATNNQAQNQNQNFLGFLLGVGSAIASGVAVSKVLHLEGEVNKIKSALLSTNKAVVSLSNGVSVLTSKVLDLKNYIDKQLLPIVNKQSCSISNIETVIEFQQKNNRLLEITREFSVNAGVTTPVSTYMLTNSELLSLINDMPITNDQKKLMSNNVQIVRQQSYSIMSIIKEEVLAYVVQLPLYGVIDTPCWKLHTSPLCTTNTKEGSNICLTRTDRGWYCDNAGSVSFFPQAETCKVQSNRVFCDTMNSLTLPSEVNLCNVDIFNPKYDCKIMTSKTDVSSSVITSLGAIVSCYGKTKCTASNKNRGIIKTFSNGCDYVSNKGVDTVSVGNTLYYVNKQEGKSLYVKGEPIINFYDPLVFPSDEFDASISQVNEKINQSLAFIRKSDELLHNVNAGKSTTNIMITTIIIVIIVILLSLIAVGLLLYCKARSTPVTLSKDQLSGINNIAFSN

SEQ ID NO: 64 - protein, 551 aa, synthetic construct
MELLILKANAITTILTAVTFCFASGQNITEEFYQSTCSAVSKGYLSALRTGWYTSVITIELSNIKENKCNGTDAKVKLIKQELDKYKNAVTELQLLMQSTPATNNRARQQQQRFLGFLLGVGSAIASGVAVSKVLHLEGEVNKIKSALLSTNKAVVSLSNGVSVLTSKVLDLKNYIDKQLLPIVNKQSCSISNIETVIEFQQKNNRLLEITREFSVNAGVTTPVSTYMLTNSELLSLINDMPITNDQKKLMSNNVQIVRQQSYSIMSIIKEEVLAYVVQLPLYGVIDTPCWKLHTSPLCTTNTKEGSNICLTRTDRGWYCDNAGSVSFFPQAETCKVQSNRVFCDTMNSLTLPSEVNLCNVDIFNPKYDCKIMTSKTDVSSSVITSLGAIVSCYGKTKCTASNKNRGIIKTFSNGCDYVSNKGVDTVSVGNTLYYVNKQEGKSLYVKGEPIINFYDPLVFPSDEFDASISQVNEKINQSLAFIRKSDELLHNVNAGKSTTNIMITTIIIVIIVILLSLIAVGLLLYCKARSTPVTLSKDQLSGINNIAFSN

SEQ ID NO: 65 - protein, 537 aa, synthetic construct
MELLILKANAITTILTAVTFCFASGQNITEEFYQSTCSAVSKGYLSALRTGWYTSVITIELSNIKENKCNGTDAKVKLIKQELDKYKNAVTELQLLMQSTPATNNQAQNELPQFMNYTLNNAQQTNVTLSKKRKRRFLGFLLGVGSAIASGVAVSKVLHLEGEVNKIKSALLSTNKAVVSLSNGVSVLTSKVLDLKNYIDKQLLPIVNKQSCSISNIETVIEFQQKNNRLLEITREFSVNAGVTTPVSTYMLTNSELLSLINDMPITNDQKKLMSNNVQIVRQQSYSIMSIIKEEVLAYVVQLPLYGVIDTPCWKLHTSPLCTTNTKEGSNICLTRTDRGWYCDNAGSVSFFPQAETCKVQSNRVFCDTMNSLTLPSEVNLCNVDIFNPKYDCKIMTSKTDVSSSVITSLGAIVSCYGKTKCTASNKNRGIIKTFSNGCDYVSNKGVDTVSVGNTLYYVNKQEGKSLYVKGEPIINFYDPLVFPSDEFDASISQVNEKINQSLAFIRKSDELLHNVNAGKSTTNGGSAGSGHHHHHH

SEQ ID NO: 66 - protein, 537 aa, synthetic construct
MELLILKANAITTILTAVTFCFASGQNITEEFYQSTCSAVSKGYLSALRTGWYTSVITIELSNIKENKCNGTDAKVKLIKQELDKYKNAVTELQLLMQSTPATNNRARRELPQFMNYTLNNAQQTNVTLSQNQNQNFLGFLLGVGSAIASGVAVSKVLHLEGEVNKIKSALLSTNKAVVSLSNGVSVLTSKVLDLKNYIDKQLLPIVNKQSCSISNIETVIEFQQKNNRLLEITREFSVNAGVTTPVSTYMLTNSELLSLINDMPITNDQKKLMSNNVQIVRQQSYSIMSIIKEEVLAYVVQLPLYGVIDTPCWKLHTSPLCTTNTKEGSNICLTRTDRGWYCDNAGSVSFFPQAETCKVQSNRVFCDTMNSLTLPSEVNLCNVDIFNPKYDCKIMTSKTDVSSSVITSLGAIVSCYGKTKCTASNKNRGIIKTFSNGCDYVSNKGVDTVSVGNTLYYVNKQEGKSLYVKGEPIINFYDPLVFPSDEFDASISQVNEKINQSLAFIRKSDELLHNVNAGKSTTNGGSAGSGHHHHHH

SEQ ID NO: 67 - protein, 528 aa, synthetic construct
MELLILKANAITTILTAVTFCFASGQNITEEFYQSTCSAVSKGYLSALRTGWYTSVITIELSNIKENKCNGTDAKVKLIKQELDKYKNAVTELQLLMQSTPATNNRARRELPRFMNYTLNNAKKTNVTLSKKRKRRSAIASGVAVSKVLHLEGEVNKIKSALLSTNKAVVSLSNGVSVLTSKVLDLKNYIDKQLLPIVNKQSCSISNIETVIEFQQKNNRLLEITREFSVNAGVTTPVSTYMLTNSELLSLINDMPITNDQKKLMSNNVQIVRQQSYSIMSIIKEEVLAYVVQLPLYGVIDTPCWKLHTSPLCTTNTKEGSNICLTRTDRGWYCDNAGSVSFFPQAETCKVQSNRVFCDTMNSLTLPSEVNLCNVDIFNPKYDCKIMTSKTDVSSSVITSLGAIVSCYGKTKCTASNKNRGIIKTFSNGCDYVSNKGVDTVSVGNTLYYVNKQEGKSLYVKGEPIINFYDPLVFPSDEFDASISQVNEKINQSLAFIRKSDELLHNVNAGKSTTNGGSAGSGHHHHHH

SEQ ID NO: 68 - protein, 531 aa, synthetic construct
MELLILKANAITTILTAVTFCFASGQNITEEFYQSTCSAVSKGYLSALRTGWYTSVITIELSNIKENKCNGTDAKVKLIKQELDKYKNAVTELQLLMQSTPATNNRARRELPRFMNYTLNNAKKTNVTLSKKRKRRGVGSAIASGVAVSKVLHLEGEVNKIKSALLSTNKAVVSLSNGVSVLTSKVLDLKNYIDKQLLPIVNKQSCSISNIETVIEFQQKNNRLLEITREFSVNAGVTTPVSTYMLTNSELLSLINDMPITNDQKKLMSNNVQIVRQQSYSIMSIIKEEVLAYVVQLPLYGVIDTPCWKLHTSPLCTTNTKEGSNICLTRTDRGWYCDNAGSVSFFPQAETCKVQSNRVFCDTMNSLTLPSEVNLCNVDIFNPKYDCKIMTSKTDVSSSVITSLGAIVSCYGKTKCTASNKNRGIIKTFSNGCDYVSNKGVDTVSVGNTLYYVNKQEGKSLYVKGEPIINFYDPLVFPSDEFDASISQVNEKINQSLAFIRKSDELLHNVNAGKSTTNGGSAGSGHHHHHH

SEQ ID NO: 69 - protein, 537 aa, synthetic construct
MELLILKANAITTILTAVTFCFASGQNITEEFYQSTCSAVSKGYLSALRTGWYTSVITIELSNIKENKCNGTDAKVKLIKQELDKYKNAVTELQLLMQSTPATNNQAQNELPQFMNYTLNNAQQTNVTLSQNQNQNFLGFLLGVGSAIASGVAVSKVLHLEGEVNKIKSALLSTNKAVVSLSNGVSVLTSKVLDLKNYIDKQLLPIVNKQSCSISNIETVIEFQQKNNRLLEITREFSVNAGVTTPVSTYMLTNSELLSLINDMPITNDQKKLMSNNVQIVRQQSYSIMSIIKEEVLAYVVQLPLYGVIDTPCWKLHTSPLCTTNTKEGSNICLTRTDRGWYCDNAGSVSFFPQAETCKVQSNRVFCDTMNSLTLPSEVNLCNVDIFNPKYDCKIMTSKTDVSSSVITSLGAIVSCYGKTKCTASNKNRGIIKTFSNGCDYVSNKGVDTVSVGNTLYYVNKQEGKSLYVKGEPIINFYDPLVFPSDEFDASISQVNEKINQSLAFIRKSDELLHNVNAGKSTTNGGSAGSGHHHHHH

SEQ ID NO: 70 - protein, 524 aa, synthetic construct
MELLILKANAITTILTAVTFCFASGQNITEEFYQSTCSAVSKGYLSALRTGWYTSVITIELSNIKENKCNGTDAKVKLIKQELDKYKNAVTELQLLMQSTPATNNQAQNELPQFMNYTLNNAQQTNVTLSQNQNQNFLGFLLGVGSAIASGVAVSKVLHLEGEVNKIKSALLSTNKAVVSLSNGVSVLTSKVLDLKNYIDKQLLPIVNKQSCSISNIETVIEFQQKNNRLLEITREFSVNAGVTTPVSTYMLTNSELLSLINDMPITNDQKKLMSNNVQIVRQQSYSIMSIIKEEVLAYVVQLPLYGVIDTPCWKLHTSPLCTTNTKEGSNICLTRTDRGWYCDNAGSVSFFPQAETCKVQSNRVFCDTMNSLTLPSEVNLCNVDIFNPKYDCKIMTSKTDVSSSVITSLGAIVSCYGKTKCTASNKNRGIIKTFSNGCDYVSNKGVDTVSVGNTLYYVNKQEGKSLYVKGEPIINFYDPLVFPSDEFDASISQVNEKINQSLAFIRKSDELLHNVNAGKSTTN

SEQ ID NO: 71 - protein, 501 aa, synthetic construct
MELLILKANAITTILTAVTFCFASGQNITEEFYQSTCSAVSKGYLSALRTGWYTSVITIELSNIKENKCNGTDAKVKLIKQELDKYKNAVTELQLLMQSTPATNNRARQQQQRFLGFLLGVGSAIASGVAVSKVLHLEGEVNKIKSALLSTNKAVVSLSNGVSVLTSKVLDLKNYIDKQLLPIVNKQSCSISNIETVIEFQQKNNRLLEITREFSVNAGVTTPVSTYMLTNSELLSLINDMPITNDQKKLMSNNVQIVRQQSYSIMSIIKEEVLAYVVQLPLYGVIDTPCWKLHTSPLCTTNTKEGSNICLTRTDRGWYCDNAGSVSFFPQAETCKVQSNRVFCDTMNSLTLPSEVNLCNVDIFNPKYDCKIMTSKTDVSSSVITSLGAIVSCYGKTKCTASNKNRGIIKTFSNGCDYVSNKGVDTVSVGNTLYYVNKQEGKSLYVKGEPIINFYDPLVFPSDEFDASISQVNEKINQSLAFIRKSDELLHNVNAGKSTTN

SEQ ID NO: 72 - DNA, 18 bp, synthetic construct
  source 1..18: mol_type = other DNA
ttggatctgcaatcgcca

SEQ ID NO: 73 - DNA, 27 bp, synthetic construct
  source 1..27: mol_type = other DNA
cttttgatcttgttcacttctccttct

SEQ ID NO: 74 - DNA, 29 bp, synthetic construct
  source 1..29: mol_type = other DNA
tggcactgctgtatctaaggtcctgcact

SEQ ID NO: 75 - protein, 4 aa, synthetic construct
LVPR

SEQ ID NO: 76 - protein, 5 aa, synthetic construct
DDDDK

SEQ ID NO: 77 - protein, 4 aa, synthetic construct
RARK

SEQ ID NO: 78 - protein, 4 aa, synthetic construct
RARQ

SEQ ID NO: 79 - protein, 4 aa, synthetic construct
QAQN

SEQ ID NO: 80 - protein, 4 aa, synthetic construct
IEGR

SEQ ID NO: 81 - protein, 4 aa, synthetic construct
RKKK

SEQ ID NO: 82 - protein, 4 aa, synthetic construct
QNQN

SEQ ID NO: 83 - protein, 4 aa, synthetic construct
QQQR

SEQ ID NO: 84 - protein, 537 aa, synthetic construct
MELLILKANAITTILTAVTFCFASGQNITEEFYQSTCSAVSKGYLSALRTGWYTSVITIELSNIKENKCNGTDAKVKLIKQELDKYKNAVTELQLLMQSTPATNNRARRELPRFMNYTLNNAKKTNVTLSKKRKRRFLGFLLGVGSAIASGVAVSKVLHLEGEVNKIKSALLSTNKAVVSLSNGVSVLTSKVLDLKNYIDKQLLPIVNKQSCSISNIETVIEFQQKNNRLLEITREFSVNAGVTTPVSTYMLTNSELLSLINDMPITNDQKKLMSNNVQIVRQQSYSIMSIIKEEVLAYVVQLPLYGVIDTPCWKLHTSPLCTTNTKEGSNICLTRTDRGWYCDNAGSVSFFPQAETCKVQSNRVFCDTMNSLTLPSEVNLCNVDIFNPKYDCKIMTSKTDVSSSVITSLGAIVSCYGKTKCTASNKNRGIIKTFSNGCDYVSNKGVDTVSVGNTLYYVNKQEGKSLYVKGEPIINFYDPLVFPSDEFDASISQVNEKINQSLAFIRKSDELLHNVNAGKSTTNGGSAGSGHHHHHH

SEQ ID NO: 85 - protein, 537 aa, synthetic construct; identical to SEQ ID NO: 66

SEQ ID NO: 86 - protein, 516 aa, synthetic construct
MELLILKANAITTILTAVTFCFASGQNITEEFYQSTCSAVSKGYLSALRTGWYTSVITIELSNIKENKCNGTDAKVKLIKQELDKYKNAVTELQLLMQSTPATNNRARQQNQQQRFLGFLLGVGSAIASGVAVSKVLHLEGEVNKIKSALLSTNKAVVSLSNGVSVLTSKVLDLKNYIDKQLLPIVNKQSCSISNIETVIEFQQKNNRLLEITREFSVNAGVTTPVSTYMLTNSELLSLINDMPITNDQKKLMSNNVQIVRQQSYSIMSIIKEEVLAYVVQLPLYGVIDTPCWKLHTSPLCTTNTKEGSNICLTRTDRGWYCDNAGSVSFFPQAETCKVQSNRVFCDTMNSLTLPSEVNLCNVDIFNPKYDCKIMTSKTDVSSSVITSLGAIVSCYGKTKCTASNKNRGIIKTFSNGCDYVSNKGVDTVSVGNTLYYVNKQEGKSLYVKGEPIINFYDPLVFPSDEFDASISQVNEKINQSLAFIRKSDELLHNVNAGKSTTNGGSAGSGHHHHHH

SEQ ID NO: 87 - protein, 537 aa, synthetic construct; identical to SEQ ID NO: 65

SEQ ID NO: 88 - protein, 537 aa, synthetic construct
MELLILKANAITTILTAVTFCFASGQNITEEFYQSTCSAVSKGYLSALRTGWYTSVITIELSNIKENKCNGTDAKVKLIKQELDKYKNAVTELQLLMQSTPATNNQAQNELQRFMNYTLNNANNTNVTLSQNQNQNFLGFLLGVGSAIASGVAVSKVLHLEGEVNKIKSALLSTNKAVVSLSNGVSVLTSKVLDLKNYIDKQLLPIVNKQSCSISNIETVIEFQQKNNRLLEITREFSVNAGVTTPVSTYMLTNSELLSLINDMPITNDQKKLMSNNVQIVRQQSYSIMSIIKEEVLAYVVQLPLYGVIDTPCWKLHTSPLCTTNTKEGSNICLTRTDRGWYCDNAGSVSFFPQAETCKVQSNRVFCDTMNSLTLPSEVNLCNVDIFNPKYDCKIMTSKTDVSSSVITSLGAIVSCYGKTKCTASNKNRGIIKTFSNGCDYVSNKGVDTVSVGNTLYYVNKQEGKSLYVKGEPIINFYDPLVFPSDEFDASISQVNEKINQSLAFIRKSDELLHNVNAGKSTTNGGSAGSGHHHHHH

SEQ ID NO: 89 - protein, 537 aa, synthetic construct; identical to SEQ ID NO: 69

SEQ ID NO: 90 - protein, 13 aa, synthetic construct
GGSAGSGHHHHHH

SEQ ID NO: 91 - protein, 45 aa, synthetic construct
TPATNNRARRELPRFMNYTLNNAKKTNVTLSKKRKRRGVGSAIAS

SEQ ID NO: 92 - protein, 51 aa, synthetic construct
TPATNNQAQNELPQFMNYTLNNAQQTNVTLSQNQNQNFLGFLLGVGSAIAS

SEQ ID NO: 93 - protein, 537 aa, synthetic construct; identical to SEQ ID NO: 69

SEQ ID NO: 94 - protein, 37 aa, Human respiratory syncytial virus
FDASISQVNEKINQSLAFIRKSDELLHHVNAGKSTTN

SEQ ID NO: 95 - protein, 52 aa, synthetic construct
FDASISQINEKINQSIAFIRKIDELLHHINAGKSTTNGSGSGDDDDKGSGSG

SEQ ID NO: 96 - protein, 71 aa, synthetic construct
FDASISQVNEKINQSLAFIRKSDELLHNVNDKIEEILSKIYHIENEIARIKKLIGEGSGSGDDDDKGSGSG

SEQ ID NO: 97 - protein, 51 aa, synthetic construct
FDASISQINEKINQILAFIRKIDELLHHINAGKSTTNGSGSGIEGRGSGSG

SEQ ID NO: 98 - protein, 70 aa, synthetic construct
FDASISQVNEKINQSLAFIRKSDELLHHVNDKIEEILSKIYHIENEIARIKKLIGEGSGSGIEGRGSGSG

SEQ ID NO: 99 - protein, 51 aa, synthetic construct
FDASISQINEKINQILAFIRKIDELLHNINAGKSTTNGSGSGLVPRGSGSG

SEQ ID NO: 100 - protein, 70 aa, synthetic construct
FDASISQVNEKINQSLAFIRKSDELLHNVNDKIEEILSKIYHIENEIARIKKLIGEGSGSGLVPRGSGSG

SEQ ID NO: 101 - DNA, 12463 bp, synthetic construct
  source 1..12463: mol_type = other DNA
ataggcggcgcatgagagaagcccagaccaattacctacccaaaatggagaaagttcacgttgacatcgaggaagacagcccattcctcagagctttgcagcggagcttcccgcagtttgaggtagaagccaagcaggtcactgataatgaccatgctaatgccagagcgttttcgcatctggcttcaaaactgatcgaaacggaggtggacccatccgacacgatccttgacattggaagtgcgcccgcccgcagaatgtattctaagcacaagtatcattgtatctgtccgatgagatgtgcggaagatccggacagattgtataagtatgcaactaagctgaagaaaaactgtaaggaaataactgataaggaattggacaagaaaatgaaggagctcgccgccgtcatgagcgaccctgacctggaaactgagactatgtgcctccacgacgacgagtcgtgtcgctacgaagggcaagtcgctgtttaccaggatgtatacgcggttgacggaccgacaagtctctatcaccaagccaataagggagttagagtcgcctactggataggctttgacaccaccccttttatgtttaagaacttggctggagcatatccatcatactctaccaactgggccgacgaaaccgtgttaacggctcgtaacataggcctatgcagctctgacgttatggagcggtcacgtagagggatgtccattcttagaaagaagtatttgaaaccatccaacaatgttctattctctgttggctcgaccatctaccacgagaagagggacttactgaggagctggcacctgccgtctgtatttcacttacgtggcaagcaaaattacacatgtcggtgtgagactatagttagttgcgacgggtacgtcgttaaaagaatagctatcagtccaggcctgtatgggaagccttcaggctatgctgctacgatgcaccgcgagggattcttgtgctgcaaagtgacagacacattgaacggggagagggtctcttttcccgtgtgcacgtatgtgccagctacattgtgtgaccaaatgactggcatactggcaacagatgtcagtgcggacgacgcgcaaaaactgctggttgggctcaaccagcgtatagtcgtcaacggtcgcacccagagaaacaccaataccatgaaaaattaccttttgcccgtagtggcccaggcatttgctaggtgggcaaaggaatataaggaagatcaagaagatgaaaggccactaggactacgagatagacagttagtcatggggtgttgttgggcttttagaaggcacaagataacatctatttataagcgcccggatacccaaaccatcatcaaagtgaacagcgatttccactcattcgtgctgcccaggataggcagtaacacattggagatcgggctgagaacaagaatcaggaaaatgttagaggagcacaaggagccgtcacctctcattaccgccgaggacgtacaagaagctaagtgcgcagccgatgaggctaaggaggtgcgtgaagccgaggagttgcgcgcagctctaccacctttggcagctgatgttgaggagcccactctggaagccgatgtagacttgatgttacaagaggctggggccggctcagtggagacacctcgtggcttgataaaggttaccagctacgatggcgaggacaagatcggctcttacgctgtgctttctccgcaggctgtactcaagagtgaaaaattatcttgcatccaccctctcgctgaacaagtcatagtgataacacactctggccgaaaagggcgttatgccgtggaaccataccatggtaaagtagtggtgccagagggacatgcaatacccgtccaggactttcaagctctgagtgaaagtgccaccattgtgtacaacgaacgtgagttcgtaaacaggtacctgcaccatattgccacacatggaggagcgctgaacactgatgaagaatattacaaaactgtcaagcccagcgagcacgacggcgaatacctgtacgacatcgacaggaaacagtgcgtcaagaaagaactagtcactgggctagggctcacaggcgagctggtggatcctcccttccatgaattcgcctacgagagtctgagaacacgaccagccgctccttaccaagtaccaaccataggggtgtatggcgtgccaggatcaggcaagtctggcatcattaaaagcgcagtcaccaaaaaagatctagtggtgagcgccaagaaagaaaactgtgcagaaattataagggacgtcaagaaaatgaaagggctggacgtcaatgccagaactgtggactcagtgctcttgaatggatgcaaacaccccgtagagaccctgtatattgacgaagcttttgcttgtcatgcaggtactctcagagcgctcatagccattataagacctaaaaaggcagtgctctgcggggatcccaaacagtgcggtttttttaacatgatgtgcctgaaagtgcattttaaccacgagatttgcacacaagtcttccacaaaagcatctctcgccgttgcactaaatctgtgacttcggtcgtctcaaccttgttttacgacaaaaaaatgagaacgacgaatccgaaagagactaagattgtgattgacactaccggcagtaccaaacctaagcaggacgatctcattctcacttgtttcagagggtgggtgaagcagttgcaaatagattacaaaggcaacgaaataatgacggcagctgcctctcaagggctgacccgtaaaggtgtgtatgccgttcggtacaaggtgaatgaaaatcctctgtacgcacccacctcagaacatgtgaacgtcctactgacccgcacggaggaccgcatcgtgtggaaaacactagccggcgacccatggataaaaacactgactgccaagtaccctgggaatttcactgccacgatagaggagtggcaagcagagcatgatgccatcatgaggcacatcttggagagaccggaccctaccgacgtcttccagaataaggcaaacgtgtgttgggccaaggctttagtgccggtgctgaagaccgctggcatagacatgaccactgaacaatggaacactgtggattattttgaaacggacaaagctcactcagcagagatagtattgaaccaactatgcgtgaggttctttggactcgatctggactccggtctattttctgcacccactgttccgttatccattaggaataatcactgggataactccccgtcgcctaacatgtacgggctgaataaagaagtggtccgtcagctctctcgcaggtacccacaactgcctcgggcagttgccactggaagagtctatgacatgaacactggtacactgcgcaattatgatccgcgcataaacctagtacctgtaaacagaagactgcctcatgctttagtcctccaccataatgaacacccacagagtgacttttcttcattcgtcagcaaattgaagggcagaactgtcctggtggtcggggaaaagttgtccgtcccaggcaaaatggttgactggttgtcagaccggcctgaggctaccttcagagctcggctggatttaggcatcccaggtgatgtgcccaaatatgacataatatttgttaatgtgaggaccccatataaataccatcactatcagcagtgtgaagaccatgccattaagcttagcatgttgaccaagaaagcttgtctgcatctgaatcccggcggaacctgtgtcagcataggttatggttacgctgacagggccagcgaaagcatcattggtgctatagcgcggcagttcaagttttcccgggtatgcaaaccgaaatcctcacttgaagagacggaagttctgtttgtattcattgggtacgatcgcaaggcccgtacgcacaatccttacaagctttcatcaaccttgaccaacatttatacaggttccagactccacgaagccggatgtgcaccctcatatcatgtggtgcgaggggatattgccacggccaccgaaggagtgattataaatgctgctaacagcaaaggacaacctggcggaggggtgtgcggagcgctgtataagaaattcccggaaagcttcgatttacagccgatcgaagtaggaaaagcgcgactggtcaaaggtgcagctaaacatatcattcatgccgtaggaccaaacttcaacaaagtttcggaggttgaaggtgacaaacagttggcagaggcttatgagtccatcgctaagattgtcaacgataacaattacaagtcagtagcgattccactgttgtccaccggcatcttttccgggaacaaagatcgactaacccaatcattgaaccatttgctgacagctttagacaccactgatgcagatgtagccatatactgcagggacaagaaatgggaaatgactctcaaggaagcagtggctaggagagaagcagtggaggagatatgcatatccgacgactcttcagtgacagaacctgatgcagagctggtgagggtgcatccgaagagttctttggctggaaggaagggctacagcacaagcgatggcaaaactttctcatatttggaagggaccaagtttcaccaggcggccaaggatatagcagaaattaatgccatgtggcccgttgcaacggaggccaatgagcaggtatgcatgtatatcctcggagaaagcatgagcagtattaggtcgaaatgccccgtcgaagagtcggaagcctccacaccacctagcacgctgccttgcttgtgcatccatgccatgactccagaaagagtacagcgcctaaaagcctcacgtccagaacaaattactgtgtgctcatcctttccattgccgaagtatagaatcactggtgtgcagaagatccaatgctcccagcctatattgttctcaccgaaagtgcctgcgtatattcatccaaggaagtatctcgtggaaacaccaccggtagacgagactccggagccatcggcagagaaccaatccacagaggggacacctgaacaaccaccacttataaccgaggatgagaccaggactagaacgcctgagccgatcatcatcgaagaggaagaagaggatagcataagtttgctgtcagatggcccgacccaccaggtgctgcaagtcgaggcagacattcacgggccgccctctgtatctagctcatcctggtccattcctcatgcatccgactttgatgtggacagtttatccatacttgacaccctggagggagctagcgtgaccagcggggcaacgtcagccgagactaactcttacttcgcaaagagtatggagtttctggcgcgaccggtgcctgcgcctcgaacagtattcaggaaccctccacatcccgctccgcgcacaagaacaccgtcacttgcacccagcagggcctgctcgagaaccagcctagtttccaccccgccaggcgtgaatagggtgatcactagagaggagctcgaggcgcttaccccgtcacgcactcctagcaggtcggtctcgagaaccagcctggtctccaacccgccaggcgtaaatagggtgattacaagagaggagtttgaggcgttcgtagcacaacaacaatgacggtttgatgcgggtgcatacatcttttcctccgacaccggtcaagggcatttacaacaaaaatcagtaaggcaaacggtgctatccgaagtggtgttggagaggaccgaattggagatttcgtatgccccgcgcctcgaccaagaaaaagaagaattactacgcaagaaattacagttaaatcccacacctgctaacagaagcagataccagtccaggaaggtggagaacatgaaagccataacagctagacgtattctgcaaggcctagggcattatttgaaggcagaaggaaaagtggagtgctaccgaaccctgcatcctgttcctttgtattcatctagtgtgaaccgtgccttttcaagccccaaggtcgcagtggaagcctgtaacgccatgttgaaagagaactttccgactgtggcttcttactgtattattccagagtacgatgcctatttggacatggttgacggagcttcatgctgcttagacactgccagtttttgccctgcaaagctgcgcagctttccaaagaaacactcctatttggaacccacaatacgatcggcagtgccttcagcgatccagaacacgctccagaacgtcctggcagctgccacaaaaagaaattgcaatgtcacgcaaatgagagaattgcccgtattggattcggcggcctttaatgtggaatgcttcaagaaatatgcgtgtaataatgaatattgggaaacgtttaaagaaaaccccatcaggcttactgaagaaaacgtggtaaattacattaccaaattaaaaggaccaaaagctgctgctctttttgcgaagacacataatttgaatatgttgcaggacataccaatggacaggtttgtaatggacttaaagagagacgtgaaagtgactccaggaacaaaacatactgaagaacggcccaaggtacaggtgatccaggctgccgatccgctagcaacagcgtatctgtgcggaatccaccgagagctggttaggagattaaatgcggtcctgcttccgaacattcatacactgtttgatatgtcggctgaagactttgacgctattatagccgagcacttccagcctggggattgtgttctggaaactgacatcgcgtcgtttgataaaagtgaggacgacgccatggctctgaccgcgttaatgattctggaagacttaggtgtggacgcagagctgttgacgctgattgaggcggctttcggcgaaatttcatcaatacatttgcccactaaaactaaatttaaattcggagccatgatgaaatctggaatgttcctcacactgtttgtgaacacagtcattaacattgtaatcgcaagcagagtgttgagagaacggctaaccggatcaccatgtgcagcattcattggagatgacaatatcgtgaaaggagtcaaatcggacaaattaatggcagacaggtgcgccacctggttgaatatggaagtcaagattatagatgctgtggtgggcgagaaagcgccttatttctgtggagggtttattttgtgtgactccgtgaccggcacagcgtgccgtgtggcagaccccctaaaaaggctgtttaagcttggcaaacctctggcagcagacgatgaacatgatgatgacaggagaagggcattgcatgaagagtcaacacgctggaaccgagtgggtattctttcagagctgtgcaaggcagtagaatcaaggtatgaaaccgtaggaacttccatcatagttatggccatgactactctagctagcagtgttaaatcattcagctacctgagaggggcccctataactctctacggctaacctgaatggactacgacatagtctagtcgacgccaccatggaactgctgatcctgaaggccaacgccatcaccaccatcctgaccgccgtgaccttctgcttcgccagcggccagaacatcaccgaggaattctaccagagcacctgcagcgccgtgagcaagggctacctgagcgccctgcggaccggctggtacaccagcgtgatcaccatcgagctgtccaacatcaaagaaaacaagtgcaacggcaccgacgccaaggtgaaactgatcaagcaggaactggacaagtacaagaacgccgtgaccgagctgcagctgctgatgcagagcacccccgccaccaacaaccgggccagaagagagctgccccggttcatgaactacaccctgaacaacgccaagaaaaccaacgtgaccctgagcaagaagcggaagcggcggttcctgggcttcctgctgggcgtgggcagcgccatcgccagcggggtggccgtgtccaaggtgctgcacctggaaggcgaggtgaacaagatcaagtccgccctgctgtccaccaacaaggccgtggtgtccctgagcaacggcgtgagcgtgctgaccagcaaggtgctggatctgaagaactacatcgacaagcagctgctgcccatcgtgaacaagcagagctgcagcatcagcaacatcgagaccgtgatcgagttccagcagaagaacaaccggctgctggaaatcacccgggagttcagcgtgaacgccggcgtgaccacccccgtgagcacctacatgctgaccaacagcgagctgctgtccctgatcaatgacatgcccatcaccaacgaccagaaaaagctgatgagcaacaacgtgcagatcgtgcggcagcagagctactccatcatgagcatcatcaaagaagaggtgctggcctacgtggtgcagctgcccctgtacggcgtgatcgacaccccctgctggaagctgcacaccagccccctgtgcaccaccaacaccaaagagggcagcaacatctgcctgacccggaccgaccggggctggtactgcgacaacgccggcagcgtgagcttcttcccccaagccgagacctgcaaggtgcagagcaaccgggtgttctgcgacaccatgaacagcctgaccctgccctccgaggtgaacctgtgcaacgtggacatcttcaaccccaagtacgactgcaagatcatgacctccaagaccgacgtgagcagctccgtgatcacctccctgggcgccatcgtgagctgctacggcaagaccaagtgcaccgccagcaacaagaaccggggcatcatcaagaccttcagcaacggctgcgactacgtgagcaacaagggcgtggacaccgtgagcgtgggcaacacactgtactacgtgaataagcaggaaggcaagagcctgtacgtgaagggcgagcccatcatcaacttctacgaccccctggtgttccccagcgacgagttcgacgccagcatcagccaggtcaacgagaagatcaaccagagcctggccttcatccggaagagcgacgagctgctgcacaatgtgaatgccggcaagagcaccaccaatatcatgatcaccacaatcatcatcgtgatcattgtgatcctgctgtctctgattgccgtgggcctgctgctgtactgcaaggcccgcagcacccctgtgaccctgtccaaggaccagctgtccggcatcaacaatatcgccttctccaactgaagtctagacggcgcgcccacccagcggccgcatacagcagcaattggcaagctgcttacatagaactcgcggcgattggcatgccgccttaaaatttttattttatttttcttttcttttccgaatcggattttgtttttaatatttcaaaaaaaaaaaaaaaaaaaaaaaaaaaaaaaaaaagggtcggcatggcatctccacctcctcgcggtccgacctgggcatccgaaggaggacgcacgtccactcggatggctaagggagagccacgtttaaaccagctccaattcgccctatagtgagtcgtattacgcgcgctcactggccgtcgttttacaacgtcgtgactgggaaaaccctggcgttacccaacttaatcgccttgcagcacatccccctttcgccagctggcgtaatagcgaagaggcccgcaccgatcgcccttcccaacagttgcgcagcctgaatggcgaatgggacgcgccctgtagcggcgcattaagcgcggcgggtgtggtggttacgcgcagcgtgaccgctacacttgccagcgccctagcgcccgctcctttcgctttcttcccttcctttctcgccacgttcgccggctttccccgtcaagctctaaatcgggggctccctttagggttccgatttagtgctttacggcacctcgaccccaaaaaacttgattagggtgatggttcacgtagtgggccatcgccctgatagacggtttttcgccctttgacgttggagtccacgttctttaatagtggactcttgttccaaactggaacaacactcaaccctatctcggtctattcttttgatttataagggattttgccgatttcggcctattggttaaaaaatgagctgatttaacaaaaatttaacgcgaattttaacaaaatattaacgcttacaatttaggtggcacttttcggggaaatgtgcgcggaacccctatttgtttatttttctaaatacattcaaatatgtatccgctcatgagacaataaccctgataaatgcttcaataatattgaaaaaggaagagtatgagtattcaacatttccgtgtcgcccttattcccttttttgcggcattttgccttcctgtttttgctcacccagaaacgctggtgaaagtaaaagatgctgaagatcagttgggtgcacgagtgggttacatcgaactggatctcaacagcggtaagatccttgagagttttcgccccgaagaacgttttccaatgatgagcacttttaaagttctgctatgtggcgcggtattatcccgtattgacgccgggcaagagcaactcggtcgccgcatacactattctcagaatgacttggttgagtactcaccagtcacagaaaagcatcttacggatggcatgacagtaagagaattatgcagtgctgccataaccatgagtgataacactgcggccaacttacttctgacaacgatcggaggaccgaaggagctaaccgcttttttgcacaacatgggggatcatgtaactcgccttgatcgttgggaaccggagctgaatgaagccataccaaacgacgagcgtgacaccacgatgcctgtagcaatggcaacaacgttgcgcaaactattaactggcgaactacttactctagcttcccggcaacaattaatagactggatggaggcggataaagttgcaggaccacttctgcgctcggcccttccggctggctggtttattgctgataaatctggagccggtgagcgtgggtctcgcggtatcattgcagcactggggccagatggtaagccctcccgtatcgtagttatctacacgacggggagtcaggcaactatggatgaacgaaatagacagatcgctgagataggtgcctcactgattaagcattggtaactgtcagaccaagtttactcatatatactttagattgatttaaaacttcatttttaatttaaaaggatctaggtgaagatcctttttgataatctcatgaccaaaatcccttaacgtgagttttcgttccactgagcgtcagaccccgtagaaaagatcaaaggatcttcttgagatcctttttttctgcgcgtaatctgctgcttgcaaacaaaaaaaccaccgctaccagcggtggtttgtttgccggatcaagagctaccaactctttttccgaaggtaactggcttcagcagagcgcagataccaaatactgttcttctagtgtagccgtagttaggccaccacttcaagaactctgtagcaccgcctacatacctcgctctgctaatcctgttaccagtggctgctgccagtggcgataagtcgtgtcttaccgggttggactcaagacgatagttaccggataaggcgcagcggtcgggctgaacggggggttcgtgcacacagcccagcttggagcgaacgacctacaccgaactgagatacctacagcgtgagctatgagaaagcgccacgcttcccgaagggagaaaggcggacaggtatccggtaagcggcagggtcggaacaggagagcgcacgagggagcttccagggggaaacgcctggtatctttatagtcctgtcgggtttcgccacctctgacttgagcgtcgatttttgtgatgctcgtcaggggggcggagcctatggaaaaacgccagcaacgcggcctttttacggttcctggccttttgctggccttttgctcacatgttctttcctgcgttatcccctgattctgtggataaccgtattaccgcctttgagtgagctgataccgctcgccgcagccgaacgaccgagcgcagcgagtcagtgagcgaggaagcggaagagcgcccaatacgcaaaccgcctctccccgcgcgttggccgattcattaatgcagctggcacgacaggtttcccgactggaaagcgggcagtgagcgcaacgcaattaatgtgagttagctcactcattaggcaccccaggctttacactttatgctcccggctcgtatgttgtgtggaattgtgagcggataacaatttcacacaggaaacagctatgaccatgattacgccaagcgcgcaattaaccctcactaaagggaacaaaagctgggtaccgggcccacgcgtaatacgactcactatag

SEQ ID NO: 102 - protein, 574 aa, Human respiratory syncytial virus
MELLILKANAITTILTAVTFCFASGQNITEEFYQSTCSAVSKGYLSALRTGWYTSVITIELSNIKENKCNGTDAKVKLIKQELDKYKNAVTELQLLMQSTPATNNRARRELPRFMNYTLNNAKKTNVTLSKKRKRRFLGFLLGVGSAIASGVAVSKVLHLEGEVNKIKSALLSTNKAVVSLSNGVSVLTSKVLDLKNYIDKQLLPIVNKQSCSISNIATVIEFQQKNNRLLEITREFSVNAGVTTPVSTYMLTNSELLSLINDMPITNDQKKLMSNNVQIVRQQSYSIMSIIKEEVLAYVVQLPLYGVIDTPCWKLHTSPLCTTNTKEGSNICLTRTDRGWYCDNAGSVSFFPQAETCKVQSNRVFCDTMNSLTLPSEVNLCNVDIFNPKYDCKIMTSKTDVSSSVITSLGAIVSCYGKTKCTASNKNRGIIKTFSNGCDYVSNKGVDTVSVGNTLYYVNKQEGKSLYVKGEPIINFYDPLVFPSDEFDASISQVNEKINQSLAFIRKSDELLHNVNAGKSTINIMITTIIIVIIVILLSLIAVGLLLYCKARSTPVTLSKDQLSGINNIAFSN

SEQ ID NO: 103 - protein, 574 aa, Human respiratory syncytial virus
MELLIHRLSAIFLTLAINALYLTSSQNITEEFYQSTCSAVSRGYFSALRTGWYTSVITIELSNIKETKCNGTDTKVKLIKQELDKYKNAVTELQLLMQNTPAANNRARREAPQYMNYTINTTKNLNVSISKKRKRRFLGFLLGVGSAIASGIAVSKVLHLEGEVNKIKNALLSTNKAVVSLSNGVSVLTSKVLDLKNYINNQLLPIVNQQSCRISNIGTVIEFQQKNSRLLEINREFSVNAGVTTPLSTYMLTNSELLSLINDMPITNDQKKLMSSNVQIVRQQSYSIMSIIKEEVLAYVVQLPIYGVIDTPCWKLHTSPLCTTNIKEGSNICLTRTDRGWYCDNAGSVSFFPQADTCKVQSNRVFCDTMNSLTLPSEVSLCNTDIFNSKYDCKIMTSKTDISSSVITSLGAIVSCYGKTKCTASNKNRGIIKTFSNGCDYVSNKGVDTVSVGNTLYYVNKLEGKNLYVKGEPIINYYDPLVFPSDEFDASISQVNEKINQSLAFIRRSDELLHNVNTGKSTTNIMITTIIIVIIVVLLSLIAIGLLLYCKAKNTPVTLSKDQLSGINNIAFSK

SEQ ID NO: 104 - protein, 574 aa, Human respiratory syncytial virus
MELLIHRLSAIFLTLAINALYLTSSQNITEEFYQSTCSAVSRGYFSALRTGWYTSVITIELSNIKETKCNGTDTKVKLIKQELDKYKNAVTELQLLMQNTPAANNRARREAPQYMNYTINTTKNLNVSISKKRKRRFLGFLLGVGSAIASGIAVSKVLHLEGEVNKIKNALLSTNKAVVSLSNGVSVLTSKVLDLKNYINNQLLPIVNQQSCRISNIETVIEFQQKNSRLLEINREFSVNAGVTTPLSTYMLTNSELLSLINDMPITNDQKKLMSSNVQIVRQQSYSIMSIIKEEVLAYVVQLPIYGVIDTPCWKLHTSPLCTTNIKEGSNICLTRTDRGWYCDNAGSVSFFPQADTCKVQSNRVFCDTMNSLTLPSEVSLCNTDIFNSKYDCKIMTSKTDISSSVITSLGAIVSCYGKTKCTASNKNRGIIKTFSNGCDYVSNKGVDTVSVGNTLYYVNKLEGKNLYVKGEPIINYYDPLVFPSDEFDASISQVNEKINQSLAFIRRSDELLHNVNTGKSTTNIMITTIIIVIIVVLLSLIAIGLLLYCKAKNTPVTLSKDQLSGINNIAFSK

SEQ ID NO: 105 - protein, 574 aa, Human respiratory syncytial virus
MELLILKANAITTILAAVTFCFASSQNITEEFYQSTCSAVSKGYLSALRTGWYTSVITIELSNIKENKCNGTDAKVKLINQELDKYKNAVTELQLLMQSTTAANNRARRELPRFMNYTLNNTKKTNVTLSKKRKRRFLGFLLGVGSAIASGIAVSKVLHLEGEVNKIKSALLSTNKAVVSLSNGVSVLTSKVLDLKNYIDKQLLPIVNKQSCRISNIETVIEFQQKNNRLLEITREFSVNAGVTTPVSTYMLTNSELLSLINDMPITNDQKKLMSNNVQIVRQQSYSIMSIIKEEVLAYVVQLPLYGVIDTPCWKLHTSPLCTTNTKEGSNICLTRTDRGWYCDNAGSVSFFPQAETCKVQSNRVFCDTMNSLTLPSEVNLCNVDIFNPKYDCKIMTSKTDVSSSVITSLGAIVSCYGKTKCTASNKNRGIIKTFSNGCDYVSNKGVDTVSVGNTLYYVNKQEGKSLYVKGEPIINFYDPLVFPSDEFDASISQVNEKINQSLAFIRKSDELLHHVNAGKSTTNIMITTIIIVIIVILLSLIAVGLLLYCKARSTPVTLSKDQLSGINNIAFSN

SEQ ID NO: 106 - protein, 574 aa, Human respiratory syncytial virus; identical to SEQ ID NO: 2

SEQ ID NO: 107 - protein, 574 aa, synthetic construct
  VARIANT 4: note = Leu or Pro
  VARIANT 6: note = His or Leu
  VARIANT 7: note = Arg or Lys
  VARIANT 8: note = Leu, Ser or Ala
  VARIANT 9: note = Ser or Asn
  VARIANT 12: note = Phe or Thr
  VARIANT 13: note = Leu or Thr
  VARIANT 14: note = Thr or Ile
  VARIANT 16: note = Ala or Thr
  VARIANT 17: note = Ile, Val or Ala
  VARIANT 18: note = Asn or Val
  VARIANT 19: note = Ala or Thr
  VARIANT 20: note = Leu or Phe
  VARIANT 21: note = Tyr or Cys
  VARIANT 22: note = Leu or Phe
  VARIANT 23: note = Thr or Ala
  VARIANT 25: note = Ser or Gly
  VARIANT 42: note = Arg or Lys
  VARIANT 45: note = Phe or Leu
  VARIANT 67: note = Thr or Asn
  VARIANT 74: note = Thr or Ala
  VARIANT 80: note = Lys or Asn
  VARIANT 99: note = Asn or Ser
  VARIANT 101: note = Pro or Thr
  VARIANT 111: note = Ala or Leu
  VARIANT 113: note = Gln or Arg
  VARIANT 114: note = Tyr or Phe
  VARIANT 124: note = Asn or Lys
  VARIANT 128: note = Ser or Thr
  VARIANT 152: note = Ile or Val
  VARIANT 169: note = Asn or Ser
  VARIANT 201: note = Asn or Lys
  VARIANT 202: note = Gln or Arg
  VARIANT 209: note = Gln or Lys
  VARIANT 213: note = Arg or Ser
  VARIANT 218: note = Gly, Glu or Ala
  VARIANT 226: note = Lys or Met
  VARIANT 228: note = Ser or Asn
  VARIANT 234: note = Asn or Thr
  VARIANT 247: note = Leu or Val
  VARIANT 276: note = Ser or Asn
  VARIANT 356: note = Asp or Glu
  VARIANT 380: note = Ser or Asn
  VARIANT 384: note = Thr or Val
  VARIANT 389: note = Ser or Pro
  VARIANT 402: note = Ile or Val
  VARIANT 462: note = Leu or Gln
  VARIANT 466: note = Asn or Ser
  VARIANT 477: note = Tyr or Phe
  VARIANT 508: note = Arg or Lys
  VARIANT 515: note = Asn or His
  VARIANT 518: note = Thr or Ala
  VARIANT 523: note = Thr or Ile
  VARIANT 537: note = Val or Ile
  VARIANT 544: note = Ile or Val
  VARIANT 553: note = Lys or Arg
  VARIANT 554: note = Asn or Ser
  VARIANT 574: note = Lys or Asn
  VARIANT 125: note = Leu or Thr
  VARIANT 121: note = Thr or Asn
  VARIANT 326: note = Ile or Thr
  VARIANT 122: note = Thr or Ala
  VARIANT 103: note = Ala or Thr
MELXIXXXXAIXXXLXXXXXXXXSXQNITEEFYQSTCSAVSXGYXSALRTGWYTSVITIELSNIKEXKCNGTDXKVKLIXQELDKYKNAVTELQLLMQXTXAXNNRARREXPXXMNYTJNXXKXXNVXJSKKRKRRFLGFLLGVGSAIASGXAVSKVLHLEGEVNKIKXALLSTNKAVVSLSNGVSVLTSKVLDLKNYIBXXLLPIVNXQSCXISNIXTVIEFQQXNXRLLEIXREFSVNAGVTTPXSTYMLTNSELLSLINDMPITNDQKKLMSXNVQIVRQQSYSIMSIIKEEVLAYVVQLPJYGVIDTPCWKLHTSPLCTTNXKEGSNICLTRTDRGWYCDNAGSVSFFPQAXTCKVQSNRVFCDTMNSLTLPSEVXLCNXDIFNXKYDCKIMTSKTDXSSSVITSLGAIVSCYGKTKCTASNKNRGIIKTFSNGCDYVSNKGVDTVSVGNTLYYVNKXEGKXLYVKGEPIINXYDPLVFPSDEFDASISQVNEKINQSLAFIRXSDELLHXVNXGKSTXNIMITTIIIVIIVXLLSLIAXGLLLYCKAXXTPVTLSKDQLSGINNIAFSX

SEQ ID NO: 108 - protein, 51 aa, Human respiratory syncytial virus
TPATNNRARRELPRFMNYTLNNAKKTNVTLSKKRKRRFLGFLLGVGSAIAS

SEQ ID NO: 109 - protein, 30 aa, synthetic construct
TPATNNRARQQNQQQRFLGFLLGVGSAIAS

SEQ ID NO: 110 - protein, 6 aa, synthetic construct
  source 1..6: note = 6xHig tag
HHHHHH

SEQ ID NO: 111 - protein, 100 aa, synthetic construct
  REGION 1..100: note = misc_feature - This sequence may encompass 3-100 Lys residues
KKKKKKKKKKKKKKKKKKKKKKKKKKKKKKKKKKKKKKKKKKKKKKKKKKKKKKKKKKKKKKKKKKKKKKKKKKKKKKKKKKKKKKKKKKKKKKKKKKKK

SEQ ID NO: 112 - protein, 50 aa, synthetic construct
IMITTIIIVIIVILLSLIAVGLLLYCKARSTPVTLSKDQLSGINNIAFSN